European Patent Specification EP 3 592 858 B1, published June 12, 2024. Title: Means and methods for lignin pyrolysis. Applicant: Universitaet des Saarlandes. The sequence listing filed with the application follows.

SEQUENCE LISTING (133 sequences)

SEQ ID NO: 1 - protein, 311 aa, P. putida
MTVKISHTADIQAFFNRVAGLDHAEGNPRFKQIILRVLQDTARLIEDLEITEDEFWHAVDYLNRLGGRNEAGLLAAGLGIEHFLDLLQDAKDAEAGLGGGTPRTIEGPLYVAGAPLAQGEARMDDGTDPGVVMFLQGQVFDADGKPLAGATVDLWHANTQGTYSYFDSTQSEFNLRRRIITDAEGRYRARSIVPSGYGCDPQGPTQECLDLLGRHGQRPAHVHFFISAPGHRHLTTQINFAGDKYLWDDFAYATRDGLIGELRFVEDAAAARDRGVQGERFAELSFDFRLQGAKSPDAEARSHRPRALQEG

SEQ ID NO: 2 - DNA, 936 bp, P. putida
atgaccgtgaaaatttcccacactgccgacattcaagccttcttcaaccgggtagctggcctggaccatgccgaaggaaacccgcgcttcaagcagatcattctgcgcgtgctgcaagacaccgcccgcctgatcgaagacctggagattaccgaggacgagttctggcacgccgtcgactacctcaaccgcctgggcggccgtaacgaggcaggcctgctggctgctggcctgggtatcgagcacttcctcgacctgctgcaggatgccaaggatgccgaagccggccttggcggcggcaccccgcgcaccatcgaaggcccgttgtacgttgccggggcgccgctggcccagggcgaagcgcgcatggacgacggcactgacccaggcgtggtgatgttccttcagggccaggtgttcgatgccgacggcaagccgttggccggtgccaccgtcgacctgtggcacgccaatacccagggcacctattcgtacttcgattcgacccagtccgagttcaacctgcgtcggcgtatcatcaccgatgccgagggccgctaccgcgcgcgctcgatcgtgccgtccgggtatggctgcgacccgcagggcccaacccaggaatgcctggacctgctcggccgccacggccagcgcccggcgcacgtgcacttcttcatctcggcaccggggcaccgccacctgaccacgcagatcaactttgctggcgacaagtacctgtgggacgactttgcctatgccacccgcgacgggctgatcggcgaactgcgttttgtcgaggatgcggcggcggcgcgcgaccgcggtgtgcaaggcgagcgctttgccgagctgtcattcgacttccgcttgcagggtgccaagtcgcctgacgccgaggcgcgaagccatcggccgcgggcgttgcaggagggctga

SEQ ID NO: 3 - protein, 304 aa, P. putida
MTVNISHTAEVQQFFEQAAGFCNAAGNPRLKRIVQRLLQDTARLIEDLDISEDEFWHAVDYLNRLGGRGEAGLLVAGLGIEHFLDLLQDAKDQEAGRVGGTPRTIEGPLYVAGAPIAQGEVRMDDGSEEGVATVMFLEGQVLDPHGRPLPGATVDLWHANTRGTYSFFDQSQSAYNLRRRIVTDAQGRYRARSIVPSGYGCDPQGPTQECLDLLGRHGQRPAHVHFFISAPGYRHLTTQINLSGDKYLWDDFAYATRDGLVGEVVFVEGPDGRHAELKFDFQLQQAQGGADEQRSGRPRALQEA

SEQ ID NO: 4 - DNA, 915 bp, P. putida
atgaccgtgaacatttcccatactgccgaggtacagcagttcttcgagcaggccgcaggcttttgtaatgcggccggcaacccacgcctcaaacgcatcgtgcagcgcctgctgcaggataccgcgcggctgatcgaagacctggacatcagcgaagacgagttctggcacgccgtcgattacctcaaccgcctgggcggtcgcggcgaagccgggttgctggtggcggggctgggcatcgaacacttcctcgacctgctgcaggatgccaaggaccaggaggcagggcgcgttggcggcaccccacgcaccatcgaaggcccgttgtacgtggctggcgcaccgattgcccaaggtgaagtgcgcatggacgacggcagcgaggagggcgtggccacggtgatgttcctggaaggccaggtgctggacccgcacggacgcccgctgccgggtgccacggtcgacctgtggcatgccaatacccgtggtacctactcgttcttcgaccaaagccagtcggcgtacaacctgcgtcggcgcatcgttaccgatgcccaggggcgctaccgcgcgcgctccatcgtgccatcgggctatggctgcgacccgcaggggccaacccaggaatgcctggacctgctgggccgtcatggccagcgcccggcgcacgtgcacttctttatctcggccccagggtaccggcacctgaccacgcagataaacctgtcgggggacaagtacctgtgggatgactttgcctatgccacacgggatgggctggtcggggaggtggtgttcgtcgaagggccggatggtcggcatgccgagctgaagttcgacttccagttgcagcaggcccagggcggtgccgatgagcagcgcagcgggcggccgcgagctttgcaggaggcctga

SEQ ID NO: 5 - DNA, 81 bp, artificial
  Promoter sequence
tgttgacaattaatcatcggcatagtatatcggcatagtataatacgacaaggtgaggaactaaaccaggaggaaaaacat

SEQ ID NO: 6 - DNA, 85 bp, artificial
  Promoter sequence
tgttgacaattaatcatcggcatagtatatcggcatagtataatacgacaaggtgaggaactaaaccaaagaggagaaattaagc

SEQ ID NO: 7 - DNA, 500 bp, artificial
  Promoter sequence
ccgcttcacagggaacaccactcaggtggtagaactggaagcggtgtcaaagcagctaagtttcagatttgattgaaaaaatttgaaaaaacgcttgacactaggacggcagacaaatagaatgccggccacatctggagggattcccgagcggtcaaaggggacggactgtaaatccgttgcgagagcttcgaaggttcgaatccttctccctccaccagttttagcgagagccgcaagctccgcgggtatagtttagtggtagaacctcagccttccaagctgatgatgcgggttcgattcccgctacccgctccaagtttgtcggattttgcacaaagtgtttcgctcttgtagctcagttggtagagcacacccttggtaagggtgaggtcagcggttcaagtccgctcaagagctccatataaacaaggcagatatgaaaatatctgcctttgttttatcagtgcaagactatttcttctgcggaggattgtatc

SEQ ID NO: 8 - DNA, 499 bp, artificial
  Promoter sequence
ggtcgagccgcccacgctggccgccctgcgcaccctgctgcaccacccactgctggccggcaaggtggaagatgccagccacttcgccgacgaagaacacctgtacagccagctgctggtggcattgatcgaagccgcgcagaaaaatcctgggctaagctcaatgcagttgatcgcacgttggcatggcaccgaacagggccgcctgctacgcgccctggcggaaaaggaatggcttatcgtggccgacaaccttgaacaacagtttttcgacactataactagcttgtccgcccgccaacgcgagcgcagcctggaacaactgctcaggaaatcacgtcaaagcgaattgaccagcgaggaaaaaacccagctcctcgccctgctgagccgaaatgttcccgcacaaacgccgacctcatctggcgcgtgaggcccatgctcgggtataatcctcggcttgttttttgcccgccaagaccttcagtggatagggtgt

SEQ ID NO: 9 - DNA, 31 bp, artificial
  Promoter sequence
tttacactttatgcttccggctcgtatggtt

SEQ ID NO: 10 - DNA, 500 bp, artificial
  Promoter sequence
aaccagtctttccatatagagcatgtgatggacggtgcctgttgatcagtgcccaaggggtgcttgatcggacacacggatcggggacaacatgaaaaaaaagaagagacatataaaaagcttttttgaagaacttataactcttaagtggataaccttctgtggataacctgcgctggcccatgaattacggggtgtacagagttttacaactttgttctgatcccgtgctgcgcttgttccaatcgtgagcgaaagctgtggatgaaaacacctgttatccacagcggagttatcaacaggctaaggggtggggttgtgcatagccctcatggtcgtttatccacagggcttattcacagaggcgaaaagccgttttggtcgataaatggctgttttgtcgtggttcctaacgtgtccacatgtggataactgaacgctcgaccggtacaatggcggtttgtttttgcctcatccggctttcaaactcaggggatatc

SEQ ID NO: 11 - DNA, 72 bp, artificial
  Promoter sequence
tgttgacaattaatcatcggcatagtatagtacgacaaggtgaggaactaaaccaaagaggagaaattaagc

SEQ ID NO: 12 - DNA, 84 bp, artificial
  Promoter sequence
tgttgacaattaatcatcggcacagtatgctggcatagtacaatacaacaaggtggggaactagaccaaagaggagaaattaag

SEQ ID NO: 13 - DNA, 70 bp, artificial
  Promoter sequence
tgttgacattaatctcggcatagtataatacgacaaggtgaggaactaaaccaaagaggagaaattaagc

SEQ ID NO: 14 - DNA, 72 bp, artificial
  Promoter sequence
tgttgacaattaatcatcggcatagtatagtatgacaaagtgaggaactgagccaaagaggagaaattaagc

SEQ ID NO: 15 - DNA, 70 bp, artificial
  Promoter sequence
tgttgacaattatctcggcatagtataatacgacaaggtgaggaactaaaccaaagaggagaaattaagc

SEQ ID NO: 16 - DNA, 85 bp, artificial
  Promoter sequence
tgttgacaattaatcatcggcatagtatattggcgtagtgtagtacggcaaggtggggaactgagccaaagaggagaaattaagc

SEQ ID NO: 17 - protein, 500 aa, Klebsiella pneumoniae
MTAPIQDLRDAIALLQQHDNQYLETDHPVDPNAELAGVYRHIGAGGTVKRPTRIGPAMMFNNIKGYPHSRILVGMHASRQRAALLLGCEASQLALEVGKAVKKPVAPVVVPASSAPCQEQIFLADDPDFDLRTLLPAPTNTPIDAGPFFCLGLALASDPVDASLTDVTIHRLCVQGRDELSMFLAAGRHIEVFRQKAEAAGKPLPITINMGLDPAIYIGACFEAPTTPFGYNELGVAGALRQRPVELVQGVSVPEKAIARAEIVIEGELLPGVRVREDQHTNSGHAMPEFPGYCGGANPSLPVIKVKAVTMRNNAILQTLVGPGEEHTTLAGLPTEASIWNAVEAAIPGFLQNVYAHTAGGGKFLGILQVKKRQPADEGRQGQAALLALATYSELKNIILVDEDVDIFDSDDILWAMTTRMQGDVSITTIPGIRGHQLDPSQTPEYSPSIRGNGISCKTIFDCTVPWALKSHFERAPFADVDPRPFAPEYFARLEKNQGS

SEQ ID NO: 18 - DNA, 1509 bp, K. pneumoniae
atgaccgcaccgattcaggatctgcgcgacgccatcgcgctgctgcaacagcatgacaatcagtatctcgaaaccgatcatccggttgaccctaacgccgagctggccggtgtttatcgccatatcggcgcgggcggcaccgtgaagcgccccacccgcatcgggccggcgatgatgtttaacaatattaagggttatccacactcgcgcattctggtgggtatgcacgccagccgccagcgggccgcgctgctgctgggctgcgaagcctcgcagctggcccttgaagtgggtaaggcggtgaaaaaaccggtcgcgccggtggtcgtcccggccagcagcgccccctgccaggaacagatctttctggccgacgatccggattttgatttgcgcaccctgcttccggcgcccaccaacacccctatcgacgccggccccttcttctgcctgggcctggcgctggccagcgatcccgtcgacgcctcgctgaccgacgtcaccatccaccgcttgtgcgtccagggccgggatgagctgtcgatgtttcttgccgccggccgccatatcgaagtgtttcgccaaaaggccgaggccgccggcaaaccgctgccgataaccatcaatatgggtctcgatccggccatctatattggcgcctgcttcgaagcccctaccacgccgttcggctataatgagctgggcgtcgccggcgcgctgcgtcaacgtccggtggagctggttcagggcgtcagcgtcccggagaaagccatcgcccgcgccgagatcgttatcgaaggtgagctgttgcctggcgtgcgcgtcagagaggatcagcacaccaatagcggccacgcgatgccggaatttcctggctactgcggcggcgctaatccgtcgctgccggtaatcaaagtcaaagcagtgaccatgcgaaacaatgcgattctgcagaccctggtgggaccgggggaagagcataccaccctcgccggcctgccaacggaagccagtatctggaatgccgtcgaggccgccattccgggctttttacaaaatgtctacgcccacaccgcgggtggcggtaagttcctcgggatcctgcaggtgaaaaaacgtcaacccgccgatgaaggccggcaggggcaggccgcgctgctggcgctggcgacctattccgagctaaaaaatattattctggttgatgaagatgtcgacatctttgacagcgacgatatcctgtgggcgatgaccacccgcatgcagggggacgtcagcattacgacaatccccggcattcgcggtcaccagctggatccgtcccagacgccggaatacagcccgtcgatccgtggaaatggcatcagctgcaagaccatttttgactgcacggtcccctgggcgctgaaatcgcactttgagcgcgcgccgtttgccgacgtcgatccgcgtccgtttgcaccggagtatttcgcccggctggaaaaaaaccagggtagcgcaaaataa

SEQ ID NO: 19 - protein, 197 aa, K. pneumoniae
MKLIIGMTGATGAPLGVALLQALRDMPEVETHLVMSKWAKTTIELETPWTAREVAALADFSHSPADQAATISSGSFRTDGMIVIPCSMKTLAGIRAGYAEGLVGRAADVVLKEGRKLVLVPREMPLSTIHLENMLALSRMGVAMVPPMPAYYNHPETVDDITNHIVTRVLDQFGLDYHKARRWNGLRTAEQFAQEIE

SEQ ID NO: 20 - DNA, 594 bp, K. pneumoniae
atgaaactgattattgggatgacgggggccaccggggcaccgcttggggtggcattgctgcaggcgctgcgcgatatgccggaggtggaaacccatctggtgatgtcgaaatgggccaaaaccaccatcgagctggaaacgccctggacggcgcgcgaagtggccgcgctggcggacttttcccacagcccggcagaccaggccgccaccatctcatccggttcatttcgtaccgacggcatgatcgttattccctgcagtatgaaaacgcttgcaggcattcgcgcgggttatgccgaaggactggtgggccacgcggcggacgtggtgctcaaagaggggcgcaagctggtgttggtcccgcgggaaatgccgctcagcacgatccatctggagaacatgctggcgctgtcccgcatgggcgtggcgatggtcccgccgatgtcagcttactacaaccacccggagacggttgacgatatcaccaatcatatcgtcacccgggtgctggatcagtttggcctcgactatcacaaagcgcgccgctggaacggcttgcgcacggcagaacaatttgcacaggagatcgaataa

SEQ ID NO: 21 - protein, 610 aa, Artificial
  Plasmid pEST1226
MTTQRNDNLEQPGRSVIFDDGLSATDTPNETNVVETEVLIVGSGPAGSSAAMFLSTQGISNIMITKYRWTANTPRAHITNQRTMEILRDAGIEDQVLAEAVPHELMGDTVYCESMAGEEIGRRPTWGTRPDRRADYELASPAMPCDIPQTLLEPIMLKNATMRGTQTQFSTEYLSHTQDDKGVSVQVLNRLTGQEYTIRAKYLIGADGARSKVAADIGGSMNITFKADLSHWRPSALDPVLGLPPRIEYRWPRRWFDRMVRPWNEWLVVWGFDINQEPPKLNDDEAIQIVRNLVGIEDLDVEILGYSLWGNNDQYATHLQKGRVCCAGDAIHKHPPSHGLGSNTSIQDSYNLCWKLACVLKGQAGPELLETYSTERAPIAKQIVTRANGSSSEYKPIFDALGVTDATTNDEFVEKLALRKENSPEGARRRAALRAALDNKDYEFNAQGTEIGQFYDSSAVITDGQKRPAMTEDPMLHHQKSTFPGLRLPHAWLGDAKEKYSTHDIAEGTRFTIFTGITGQAWADAAVRVAERLGIDLKAVVIGEGQPVQDLYGDWLRQREVDEDGVILVRPDKHIGWRAQSMVADPETALFDVLSALLHTKQTGSSHLRV

SEQ ID NO: 22 - DNA, 1833 bp, Artificial
  Plasmid pEST1226
atgactacacagcgtaatgataatcttgagcagccgggccgtagcgtcatttttgatgatgggctgagcgcaactgataccccaaatgagaccaacgtagttgaaactgaggtgttaattgtcggttcaggccctgctggcagctccgcagcaatgttcctgtcgacccagggcattagcaacattatgatcaccaaataccgttggactgcgaataccccccgtgcgcatatcactaaccagcgcaccatggaaattttacgcgacgctggtattgaggatcaggttttagcagaagcagtcccccatgaacttatgggtgacacagtctattgtgagtcaatggccggcgaagaaattggccgccggccaacttggggcacacgacctgaccgccgcgctgactatgagctggcatctccagcgatgccttgcgatatcccgcaaaccttgcttgagcccattatgctcaaaaatgccaccatgcgtggcacgcaaacacagttctccactgagtatttaagccacacccaagacgataagggtgtcagcgtgcaagtactcaaccgtctgaccggtcaagaatataccattcgcgccaaatacctgattggtgctgatggtgcgcgctccaaagtggctgcggatatcggcggctcgatgaatatcacctttaaagcagacttgtcccactggcgcccatcggccctcgatcctgtattgggtcttccgcccaggatcgaatatcggtggcctcggcgctggtttgatcgcatggtgcggccatggaatgaatggctggtggtctggggttttgatatcaatcaagagccacccaagctcaatgacgatgaagctattcaaatcgtgcgtaatctagtgggtatcgaggatcttgatgtggaaatccttggctactcactctggggcaataatgaccagtacgccacgcatctacagaaaggccgcgtatgctgtgccggtgatgcaatccataagcatccgcccagtcacggcctgggttctaatacgtcaatccaagactcctacaacctgtgctggaagttggcctgtgtactcaaagggcaggcggggcctgaactgttagaaacctattccaccgagcgtgcacccatcgccaagcagattgtgacgcgtgccaacggctcgagcagtgaatataagccgatttttgacgctttaggcgttaccgatgcgacaaccaacgatgagtttgtagaaaagcttgccttgcgtaaggaaaattcgcctgaaggtgctcgccgtcgagcagcattgcgtgcggcgctggacaataaggattatgagtttaacgcccaaggcactgaaattggtcagttctacgactcatcagcagtgattactgatggtcaaaaacgcccagcaatgaccgaggatcctatgctacaccaccagaaatcgacctttcctggactacgcctaccccatgcatggctaggtgatgcgaaagagaaatactccacccatgatattgcggagggcactcgcttcacgattttcactggtatcaccggtcaagcttgggctgatgcagcagttcgcgttgctgagcgtttgggcatcgacttgaaggccgtggtgattggtgaagggcagccggtacaagacctctatggcgattggttacgccagcgtgaagtggacgaggacggtgtgatcttggtgcgcccagataaacatattggttggcgtgcccagagtatggtcgcagatccagagactgcattatttgatgtactctcagcgctgctgcataccaagcaaaccggctcttcgcatttaagggtgtag

SEQ ID NO: 23 - protein, 521 aa, P. putida
MSEQNNAVLPKGVTQGEFNKAVQKFRALLGDDNVLVESDQLVPYNKIMMPVENAAHAPSAAVTATTVEQVQGVVKICNEHKIPIWTISTGRNFGYGSAAPVQRGQVILDLKKMNKIIKIDPEMCYALVEPGVTFGQMYDYIQENNLPVMLSFSAPSAIAGPVGNTMDRGVGYTPYGEHFMMQCGMEVVLANGDVYRTGMGGVPGSNTWQIFKWGYGPTLDGMFTQANYGICTKMGFWLMPKPPVFKPFEVIFEDEADIVEIVDALRPLRMSNTIPNSVVIASTLWEAGSAHLTRAQYTTEPGHTPDSVIKQMQKDTGMGAWNLYAALYGTQEQVDVNWKIVTDVFKKLGKGRIVTQEEAGDTQPFKYRAQLMSGVPNLQEFGLYNWRGGGGSMWFAPVSEARGSECKKQAAMAKRVLHKYGLDYVAEFIVAPRDMHHVIDVLYDRTNPEETKRADACFNELLDEFEKEGYAVYRVNTRFQDRVAQSYGPVKRKLEHAIKRAVDPNNILAPGRSGIDLNNDF

SEQ ID NO: 24 - DNA, 1566 bp, P. putida
atgtccgagcaaaacaatgctgtgttgcccaaaggggtaacgcagggcgagttcaacaaggcggtgcagaaattccgcgccttgctgggtgacgataatgtattggtcgaatccgaccagttggtgccttacaacaagatcatgatgccggtcgagaatgcggctcatgccccctcggccgccgtcaccgcgaccaccgtcgagcaggtgcagggtgtagtcaagatctgtaacgaacacaaaattccgatctggaccatctccactgggcgcaacttcggttacgggtccgccgcgccggtgcagcgcggtcaggtaatccttgacctgaagaagatgaacaagatcatcaagatcgacccggaaatgtgctatgcgctggtcgagccgggggttaccttcggtcagatgtatgactacatccaggaaaacaacctgccggtgatgctgtcgttctcggcaccctcggcgattgccggcccggtcggcaataccatggaccgaggcgtgggctacaccccctacggcgaacacttcatgatgcagtgcggcatggaagtggtgctggccaacggtgacgtttaccgcaccggcatgggtggcgtgcctggcagcaacacctggcagattttcaaatggggctatggtccgaccctggatggcatgttcactcaggccaactatggcatttgcaccaagatgggcttctggctgatgcccaagccgcccgtgttcaagccgttcgaagtgatcttcgaggacgaggcggacatcgtcgagatcgtcgatgcactgcgcccgctgcgcatgagcaacaccatccccaactcggtggtaatcgccagcaccttgtgggaagccggcagtgcgcacctgacccgcgcccagtacaccaccgagccgggccacacgccggatagcgtgatcaagcagatgcagaaagacaccggcatgggtgcctggaacctctacgctgcgctgtacggtacccaggaacaggtcgacgtaaactggaagatcgtaactgacgtcttcaagaaacttggcaagggccgtatcgtcacccaggaagaggcgggtgacacccagccgttcaaataccgtgcccagctgatgtccggcgtgcccaacctgcaggaattcggcctgtacaactggcgtgggggcggtggctccatgtggttcgcgccggtcagcgaggcgcgtggcagcgagtgcaagaagcaggcggccatggccaagcgcgttctgcacaagtacggcctggattatgtggccgagttcatcgtggcgccgcgcgacatgcaccacgtcatcgacgtgctctacgaccgcaccaatcctgaggaaaccaagcgcgccgacgcctgcttcaatgagctgctggatgagttcgagaaggaaggctatgcggtgtatcgggtgaacacccgcttccaggatcgcgtggcgcagagctatggcccggtcaagcgcaagctggagcatgccatcaagcgtgcggtggacccgaacaacatcctcgctccgggccgctcgggcatcgacctcaataacgatttctga

SEQ ID NO: 25 - protein, 113 aa, P. putida
MTFPFSGAAVKRMLVTGVVLPFGLLVAAGQAQADSQWGSGKNLYDKVCGHCHKPEVGVGPVLEGRGLPEAYIKDIVRNGFRAMPAFPASYVDDESLTQVAEYLSSLPAPAAQP

SEQ ID NO: 26 - DNA, 342 bp, P. putida
atgacatttccctttagcggcgcagctgtgaaacggatgctcgtgactggagttgtgcttccctttggtctgctggtcgcagcgggacaggcgcaggccgacagccagtggggcagtggcaagaacctgtatgacaaggtttgtggccattgccacaagcccgaagtcggggtagggccggttcttgagggtcgcggcctgccggaagcctacatcaaggacattgtgcgcaacggcttccgtgccatgccggcattcccggcgtcttatgttgatgacgaatcccttactcaggtggctgaatacctgtcgagcctgccggccccagcggctcagccttga

SEQ ID NO: 27 - protein, 373 aa, Pseudomonas putida
MTSVLIEHIDAIIVDLPTIRPHKLAMHTMQQQTLVVLRLRCSDGVEGIGEATTIGGLAYGYESPEGIKANIDAYLAPALIGLPADNINAAMLKLDKLAKGNTFAKSGIESALLDAQGKRLGLPVSELLGGRVRDSLEVAWTLASGDTARDIAEAQHMLDIRRHRVFKLKIGANPVAQDLKHVVAIKRELGDSASVRVDVNQYWDESQAIRACQVLGDNGIDLIEQPISRINRAGQVRLNQRSPAPIMADESIESVEDAFSLAADGAASIFALKIAKNGGPRAVLRTAQIAEAAGIALYGGTMLEGSIGTLASAHAFLTLRQLTWGTELFGPLLLTEEIVNEPPQYRDFQLHIPHTPGLGLTLDEQRLARFARR

SEQ ID NO: 28 - DNA, 1122 bp, P. putida
atgacaagcgtgctgattgaacacatagatgcaattatcgtcgatctcccgaccattcgcccgcacaagctggcgatgcacaccatgcagcagcagaccctggtggtattgcgactgcgctgcagcgatggcgtggaaggcatcggtgaagccaccaccatcggtggcctggcgtatggctacgaaagccccgaagggatcaaggccaacatcgacgcgtacctcgccccagcgttgattggcctgccggcagacaacatcaatgccgccatgctcaagctggacaagctggccaagggcaacaccttcgccaagtccggcatcgaaagcgccttgctcgacgcccagggcaaacgcctgggcctgccggtcagcgaactgctgggtggccgcgtgcgtgacagcctggaagtggcctggaccctggccagcggcgacaccgcccgcgacatcgccgaagcacagcacatgctggacattcgccggcaccgcgtgttcaagctgaaaatcggcgccaacccggtggcgcaggacctcaagcacgtggtcgcgatcaagcgcgagctgggtgacagcgccagcgtgcgggtcgacgtcaaccagtactgggacgagtcccaggccatccgcgcctgccaggtattgggcgacaacggcatcgacctgatcgagcagccgatttcgcgcatcaaccgcgctggccaggtgcgcctgaaccagcgcagtccggctccgatcatggccgatgagtcgatcgaaagcgtcgaggacgccttcagcctggccgccgacggcgccgccagcatcttcgccctgaaaatcgccaagaatggtggcccgcgcgcggttctgcgcactgcacagatcgccgaggccgctggcatcgccttgtacggcggcaccatgctcgaaggttcgatcggcaccctggcttcggctcatgcattcctcaccctgcgccagctcacctggggtacagagctgttcgggccgctgctgctgaccgaggagatcgtcaacgagccgccgcaataccgcgacttccagctgcacatcccccacaccccaggcctgggcctgacgttggacgaacagcgcctggcgcgcttcgcccgtcgctga

SEQ ID NO: 29 - protein, 96 aa, P. putida
MLFHVKMTVKLPVDMDPAKAAQLKADEKELAQRLQREGIWRHLWRIAGHYANYSVFDVPSVEALHDTLMQLPLFPYMDIEVDGLCRHPSSIHSDDR

SEQ ID NO: 30 - DNA, 291 bp, P. putida
atgttgttccacgtgaagatgaccgtgaagctgccggtcgacatggacccggccaaggccgcccagctcaaggccgacgaaaaggaactggcccagcgcctgcagcgcgaaggcatctggcgtcacctgtggcgcattgccgggcattacgccaactacagcgtgttcgatgtgcccagcgtcgaggcattgcatgacacgctgatgcagctgccgctgttcccgtacatggatatcgaggtcgacggcctgtgtcggcatccctcgtctattcacagcgacgatcgctga

SEQ ID NO: 31 - protein, 450 aa, P. putida
MSNQLFDAYFTAPAMREIFSDRGRLQGMLDFEAALARAEASAGLVPHSAVAAIEAACQAERYDVGALANAIATAGNSAIPLVKALGKVIATGVPEAERYVHLGATSQDAMDTGLVLQLRDALDLIEADLGKLADTLSQQALKHADTPLVGRTWLQHATPVTLGMKLAGVLGALTRHRQRLQELRPRLLVLQFGGASGSLAALGSKAMPVAEALAEQLKLTLPEQPWHTQRDRLVEFASVLGLVAGSLGKFGRDISLLMQTEAGEVFEPSAPGKGGSSTMPHKRNPVGAAVLIGAATRVPGLLSTLFAAMPQEHERSLGLWHAEWETLPDICCLVSGALRQAQVIAEGMEVDAARMRRNLDLTQGLVLAEAVSIVLAQRLGRDRAHHLLEQCCQRAVAEQRHLRAVLGDEPQVSAELSGEELDRLLDPAHYLGQARVWVARAVSEHQRFTA

SEQ ID NO: 32 - DNA, 1353 bp, P. putida
atgagcaaccaactgttcgacgcctatttcaccgcgccggccatgcgcgagattttctccgaccgaggccgcctgcagggcatgctggatttcgaagccgcgcttgcccgagccgaagcctctgccggtttggtcccgcacagcgcggtagcggccatcgaggcggcatgccaggccgagcgctatgacgttggcgcgctggccaatgccatcgccaccgcgggcaactcggccattccgctggtgaaagcgttgggcaaggtgatcgccaccggcgtgccagaggctgagcgctatgtgcaccttggggccaccagccaggatgcgatggataccggtctggttctgcagctgcgcgatgccctcgatttgatcgaggccgacctcggcaagctggccgataccctgtcgcagcaggccttgaagcacgccgatacgcccttggtgggtcgtacctggttgcaacacgccaccccggtgaccctgggcatgaaactggccggtgtactgggtgctttgacccgccaccgtcagcgcctgcaggaactgcgcccgcgccttctggtcctgcagttcggcggtgcctcgggcagcctggcggcgctgggcagcaaggcgatgccggtggccgaagcgctggccgaacagctcaagctgaccctgcccgagcagccctggcacacccagcgcgaccgcctggtggagtttgcctcggtattgggcctggttgccggcagcctgggcaagttcggccgtgatatcagcttgctgatgcaaaccgaggcgggggaggtgtttgagccttctgcgccgggcaagggtggttcttcgaccatgccacacaagcgcaacccggtgggtgccgccgtgttgatcggtgccgcgacccgcgtgccgggcctgctgtcgacgctgttcgcagccatgcctcaggagcacgaacgcagcctgggcctatggcatgccgagtgggaaaccctgccggatatctgctgcctggtctctggcgccctgcgccaggctcaagtgattgccgagggcatggaggtggatgccgcgcgcatgcgccgtaacctcgacctgacccaaggcctggtgctggccgaagcggtgagcatcgtcctcgcccagcgtctgggtcgcgaccgtgcccaccacctgctggaacaatgctgccaacgcgcggtggccgaacagcggcacctgcgtgccgtgctgggtgacgagccgcaggtcagcgccgagctgtctggcgaagaactcgatcgcctgctcgaccctgcccattacctgggccaggcccgcgtctgggtggcgcgcgccgtgtccgaacatcaacgtttcactgcctga

SEQ ID NO: 33 - DNA, 1509 bp, Artificial
  aroY codon optimized
atgaccgcgccgatccaggacctgcgcgatgcgatcgcgctgttgcagcagcatgacaaccagtacctggaaaccgatcatccggtcgatcccaacgccgaactggcgggcgtctaccgccacatcggtgccggcgggaccgtgaagcgtcccacccggatcggtcccgccatgatgttcaacaacatcaagggctatccccattcccgcattctggtcggcatgcacgcgagtcgccaacgggccgctctgctgttgggctgcgaagccagccaactggcactggaggtggggaaagcggtcaagaagccagtagccccggtagtggtgcccgccagtagcgcaccttgtcaggaacagatcttcctggcggatgacccggacttcgacctgcgcaccttgctgcctgccccgacgaatacgccgatcgatgctggcccgttcttctgcctgggcctcgccctcgcgagcgatccagtggacgcaagcctcaccgatgtcaccattcaccgcctgtgtgtgcaggggcgcgacgaactgagcatgttcctcgcagctggtcgccacatcgaagtgttccgccaaaaggccgaggccgcgggcaaacccctgcccattaccatcaacatgggcctggacccggccatctacatcggcgcttgctttgaggctccgaccactccgttcggctacaacgaactcggcgtagccggcgccttgcgccaacgcccagtagagctggttcagggtgtgtcggtgcccgagaaagcgattgcccgtgccgagatcgtcatcgaaggcgaactgctccctggcgttcgcgtccgcgaggaccagcacaccaattcgggccatgcgatgccagagtttccaggctattgcggtggcgccaatccgagcttgccggtgatcaaggtcaaagccgtgaccatgcggaacaacgcgatcctgcagaccctggtgggccctggggaggagcacaccactctggcggggctgccgaccgaagccagcatctggaatgcggtggaagctgccatccccggcttcctgcagaacgtctacgcccacactgcgggtggcggcaagttcctggggattctgcaggttaagaagcggcaaccggccgacgaaggccgccagggtcaggccgccttgctggcactggccacctactccgaactgaagaacatcatcctggtggacgaggatgtggacatcttcgacagcgacgacatcctgtgggccatgacgacccgcatgcagggtgacgtgtcgatcaccaccattccgggcattcgcggtcaccagctggatcctagccagacgcccgagtattcgccgagcatccgcggcaacggcatctcctgcaagacgatcttcgactgcaccgtgccgtgggccctgaagagccactttgagcgtgcaccgtttgccgacgtcgacccgcgtccgttcgccccagagtacttcgcacgtttggagaagaaccagggctcggccaaatga

SEQ ID NO: 34 - DNA, 594 bp, Artificial
  kpdB codon optimized
atgaagctgatcatcgggatgaccggtgccactggcgctcccttgggtgttgccctcctgcaggcactgcgcgacatgccagaggtcgaaacccacctggtgatgtccaagtgggccaagacgaccattgagctggaaaccccgtggacggctcgcgaagtggcagcgttggcggacttcagccacagtccagccgatcaagcggccaccatctcgagcgggagctttcggaccgatggcatgatcgtcatcccgtgctcgatgaaaaccctggccggtattcgcgcaggctatgccgaaggcctggtcggccatgccgccgatgtggtcctgaaggagggccgtaagctcgtgctggtgcctcgcgagatgcccctgtccacgatccacctggagaacatgctggccttgagccgcatgggcgtagccatggttccgccgatgagcgcctactacaaccatccggaaaccgtggacgacatcaccaaccacatcgtgacccgggtactcgaccagttcggcctggactaccacaaagcgcgccgctggaatggcctgcgtaccgcggaacagttcgcgcaggagatcgagtga

SEQ ID NO: 35 - DNA, 2193 bp, Artificial
  Artificial construct
tgttgacaattaatcatcggcatagtatagtacgacaaggtgaggaactaaaccaaagaggagaaattaagcatgaccgcaccgattcaggatctgcgcgacgccatcgcgctgctgcaacagcatgacaatcagtatctcgaaaccgatcatccggttgaccctaacgccgagctggccggtgtttatcgccatatcggcgcgggcggcaccgtgaagcgccccacccgcatcgggccggcgatgatgtttaacaatattaagggttatccacactcgcgcattctggtgggtatgcacgccagccgccagcgggccgcgctgctgctgggctgcgaagcctcgcagctggcccttgaagtgggtaaggcggtgaaaaaaccggtcgcgccggtggtcgtcccggccagcagcgccccctgccaggaacagatctttctggccgacgatccggattttgatttgcgcaccctgcttccggcgcccaccaacacccctatcgacgccggccccttcttctgcctgggcctggcgctggccagcgatcccgtcgacgcctcgctgaccgacgtcaccatccaccgcttgtgcgtccagggccgggatgagctgtcgatgtttcttgccgccggccgccatatcgaagtgtttcgccaaaaggccgaggccgccggcaaaccgctgccgataaccatcaatatgggtctcgatccggccatctatattggcgcctgcttcgaagcccctaccacgccgttcggctataatgagctgggcgtcgccggcgcgctgcgtcaacgtccggtggagctggttcagggcgtcagcgtcccggagaaagccatcgcccgcgccgagatcgttatcgaaggtgagctgttgcctggcgtgcgcgtcagagaggatcagcacaccaatagcggccacgcgatgccggaatttcctggctactgcggcggcgctaatccgtcgctgccggtaatcaaagtcaaagcagtgaccatgcgaaacaatgcgattctgcagaccctggtgggaccgggggaagagcataccaccctcgccggcctgccaacggaagccagtatctggaatgccgtcgaggccgccattccgggctttttacaaaatgtctacgcccacaccgcgggtggcggtaagttcctcgggatcctgcaggtgaaaaaacgtcaacccgccgatgaaggccggcaggggcaggccgcgctgctggcgctggcgacctattccgagctaaaaaatattattctggttgatgaagatgtcgacatctttgacagcgacgatatcctgtgggcgatgaccacccgcatgcagggggacgtcagcattacgacaatccccggcattcgcggtcaccagctggatccgtcccagacgccggaatacagcccgtcgatccgtggaaatggcatcagctgcaagaccatttttgactgcacggtcccctgggcgctgaaatcgcactttgagcgcgcgccgtttgccgacgtcgatccgcgtccgtttgcaccggagtatttcgcccggctggaaaaaaaccagggtagcgcaaaataaaaagaggagaaattaagcatgaagctgatcatcgggatgaccggtgccactggcgctcccttgggtgttgccctcctgcaggcactgcgcgacatgccagaggtcgaaacccacctggtgatgtccaagtgggccaagacgaccattgagctggaaaccccgtggacggctcgcgaagtggcagcgttggcggacttcagccacagtccagccgatcaagcggccaccatctcgagcgggagctttcggaccgatggcatgatcgtcatcccgtgctcgatgaaaaccctggccggtattcgcgcaggctatgccgaaggcctggtcggccatgccgccgatgtggtcctgaaggagggccgtaagctcgtgctggtgcctcgcgagatgcccctgtccacgatccacctggagaacatgctggccttgagccgcatgggcgtagccatggttccgccgatgagcgcctactacaaccatccggaaaccgtggacgacatcaccaaccacatcgtgacccgggtactcgaccagttcggcctggactaccacaaagcgcgccgctggaatggcctgcgtaccgcggaacagttcgcgcaggagatcgagtga

SEQ ID NO: 36 - DNA, 3947 bp, Artificial
  artificial construct
ttgttgacaattaatcatcggcatagtatatcggcatagtataatacgacaaggtgaggaactaaacccctaggttaaagaggagaaattaagcatgtccgagcaaaacaatgctgtgttgcccaaaggggtaacgcagggcgagttcaacaaggcggtgcagaaattccgcgccttgctgggtgacgataatgtattggtcgaatccgaccagttggtgccttacaacaagatcatgatgccggtcgagaatgcggctcatgccccctcggccgccgtcaccgcgaccaccgtcgagcaggtgcagggtgtagtcaagatctgtaacgaacacaaaattccgatctggaccatctccactgggcgcaacttcggttacgggtccgccgcgccggtgcagcgcggtcaggtaatccttgacctgaagaagatgaacaagatcatcaagatcgacccggaaatgtgctatgcgctggtcgagccgggggttaccttcggtcagatgtatgactacatccaggaaaacaacctgccggtgatgctgtcgttctcggcaccctcggcgattgccggcccggtcggcaataccatggaccgaggcgtgggctacaccccctacggcgaacacttcatgatgcagtgcggcatggaagtggtgctggccaacggtgacgtttaccgcaccggcatgggtggcgtgcctggcagcaacacctggcagattttcaaatggggctatggtccgaccctggatggcatgttcactcaggccaactatggcatttgcaccaagatgggcttctggctgatgcccaagccgcccgtgttcaagccgttcgaagtgatcttcgaggacgaggcggacatcgtcgagatcgtcgatgcactgcgcccgctgcgcatgagcaacaccatccccaactcggtggtaatcgccagcaccttgtgggaagccggcagtgcgcacctgacccgcgcccagtacaccaccgagccgggccacacgccggatagcgtgatcaagcagatgcagaaagacaccggcatgggtgcctggaacctctacgctgcgctgtacggtacccaggaacaggtcgacgtaaactggaagatcgtaactgacgtcttcaagaaacttggcaagggccgtatcgtcacccaggaagaggcgggtgacacccagccgttcaaataccgtgcccagctgatgtccggcgtgcccaacctgcaggaattcggcctgtacaactggcgtgggggcggtggctccatgtggttcgcgccggtcagcgaggcgcgtggcagcgagtgcaagaagcaggcggccatggccaagcgcgttctgcacaagtacggcctggattatgtggccgagttcatcgtggcgccgcgcgacatgcaccacgtcatcgacgtgctctacgaccgcaccaatcctgaggaaaccaagcgcgccgacgcctgcttcaatgagctgctggatgagttcgagaaggaaggctatgcggtgtatcgggtgaacacccgcttccaggatcgcgtggcgcagagctatggcccggtcaagcgcaagctggagcatgccatcaagcgtgcggtggacccgaacaacatcctcgctccgggccgctcgggcatcgacctcaataacgatttctgaaaagaggagaaattaagcatgacatttccctttagcggcgcagctgtgaaacggatgctcgtgactggagttgtgcttccctttggtctgctggtcgcagcgggacaggcgcaggccgacagccagtggggcagtggcaagaacctgtatgacaaggtttgtggccattgccacaagcccgaagtcggggtagggccggttcttgagggtcgcggcctgccggaagcctacatcaaggacattgtgcgcaacggcttccgtgccatgccggcattcccggcgtcttatgttgatgacgaatcccttactcaggtggctgaatacctgtcgagcctgccggccccagcggctcagccttgattgttgacaattaatcatcggcatagtatatcggcatagtataatacgacaaggtgaggaactaaacccctaggttaaagaggagaaattaagcatgactacacagcgtaatgataatcttgagcagccgggccgtagcgtcatttttgatgatgggctgagcgcaactgataccccaaatgagaccaacgtagttgaaactgaggtgttaattgtcggttcaggccctgctggcagctccgcagcaatgttcctgtcgacccagggcattagcaacattatgatcaccaaataccgttggactgcgaataccccccgtgcgcatatcactaaccagcgcaccatggaaattttacgcgacgctggtattgaggatcaggttttagcagaagcagtcccccatgaacttatgggtgacacagtctattgtgagtcaatggccggcgaagaaattggccgccggccaacttggggcacacgacctgaccgccgcgctgactatgagctggcatctccagcgatgccttgcgatatcccgcaaaccttgcttgagcccattatgctcaaaaatgccaccatgcgtggcacgcaaacacagttctccactgagtatttaagccacacccaagacgataagggtgtcagcgtgcaagtactcaaccgtctgaccggtcaagaatataccattcgcgccaaatacctgattggtgctgatggtgcgcgctccaaagtggctgcggatatcggcggctcgatgaatatcacctttaaagcagacttgtcccactggcgcccatcggccctcgatcctgtattgggtcttccgcccaggatcgaatatcggtggcctcggcgctggtttgatcgcatggtgcggccatggaatgaatggctggtggtctggggttttgatatcaatcaagagccacccaagctcaatgacgatgaagctattcaaatcgtgcgtaatctagtgggtatcgaggatcttgatgtggaaatccttggctactcactctggggcaataatgaccagtacgccacgcatctacagaaaggccgcgtatgctgtgccggtgatgcaatccataagcatccgcccagtcacggcctgggttctaatacgtcaatccaagactcctacaacctgtgctggaagttggcctgtgtactcaaagggcaggcggggcctgaactgttagaaacctattccaccgagcgtgcacccatcgccaagcagattgtgacgcgtgccaacggctcgagcagtgaatataagccgatttttgacgctttaggcgttaccgatgcgacaaccaacgatgagtttgtagaaaagcttgccttgcgtaaggaaaattcgcctgaaggtgctcgccgtcgagcagcattgcgtgcggcgctggacaataaggattatgagtttaacgcccaaggcactgaaattggtcagttctacgactcatcagcagtgattactgatggtcaaaaacgcccagcaatgaccgaggatcctatgctacaccaccagaaatcgacctttcctggactacgcctaccccatgcatggctaggtgatgcgaaagagaaatactccacccatgatattgcggagggcactcgcttcacgattttcactggtatcaccggtcaagcttgggctgatgcagcagttcgcgttgctgagcgtttgggcatcgacttgaaggccgtggtgattggtgaagggcagccggtacaagacctctatggcgattggttacgccagcgtgaagtggacgaggacggtgtgatcttggtgcgcccagataaacatattggttggcgtgcccagagtatggtcgcagatccagagactgcattatttgatgtactctcagcgctgctgcataccaagcaaaccggctcttcgcatttaagggtgtag

SEQ ID NO: 37 - DNA, 23 bp, artificial
  primer
ccattcaggctgcgcaactgttg

SEQ ID NO: 38 - DNA, 22 bp, artificial
  primer
ctttacactttatgcttccggc

SEQ ID NO: 39 - DNA, 20 bp, artificial
  primer
ggacgcttcgctgaaaacta

SEQ ID NO: 40 - DNA, 20 bp, artificial
  primer
aacgtcgtgactgggaaaac

SEQ ID NO: 41 - DNA, 24 bp, artificial
  primer
ggcacatcgaacacgctgtagttg

SEQ ID NO: 42 - DNA, 24 bp, artificial
  primer
cctccagggtatggtgggagattc

SEQ ID NO: 43 - DNA, 34 bp, artificial
  primer
tgaacgcttcgccagccaactaccttcgccagcc

SEQ ID NO: 44 - DNA, 28 bp, artificial
  primer
gctcgatacccaggccagcaggccagca

SEQ ID NO: 45 - DNA, 28 bp, artificial
  primer
catatgtgttgccaggtcccgtcaggtc

SEQ ID NO: 46 - DNA, 33 bp, artificial
  primer
aaaaacatatgcagctcaaggccgacgaaaagg

SEQ ID NO: 47 - DNA, 40 bp, artificial
  primer
tgaattcgagctcggtaccctgggcgatgtgcagcagctc

SEQ ID NO: 48 - DNA, 41 bp, artificial
  primer
cgatgattaattgtcaacaacgtgcttacctcgtattgttc

SEQ ID NO: 49 - DNA, 42 bp, artificial
  primer
ttaaagaggagaaattaagcatgaccgtgaaaatttcccaca

SEQ ID NO: 50 - DNA, 41 bp, artificial
  primer
gtcgactctagaggatcccctcgaagtacgaataggtgccc

SEQ ID NO: 51 - DNA, 51 bp, artificial
  primer
gcctgacaagaacaatacgaggtaagcacgttgttgacaattaatcatcgg

SEQ ID NO: 52 - DNA, 57 bp, artificial
  primer
gtcggcagtgtgggaaattttcacggtcatgcttaatttctcctctttaacctaggg

SEQ ID NO: 53 - DNA, 4389 bp, artificial
  pEMG-deltacatB catC
  misc_feature (3555)..(3555): n is a, c, g, or t
gccggcgtcccggaaaacgattccgaagcccaacctttcatagaaggcggcggtggaatcgaaatctcgtgatggcaggttgggcgtcgcttggtcggtcatttcgaaccccagagtcccgctcagaagaactcgtcaagaaggcgatagaaggcgatgcgctgcgaatcgggagcggcgataccgtaaagcacgaggaagcggtcagcccattcgccgccaagctcttcagcaatatcacgggtagccaacgctatgtcctgatagcggtccgccacacccagccggccacagtcgatgaatccagaaaagcggccattttccaccatgatattcggcaagcaggcatcgccatgggtcacgacgagatcctcgccgtcgggcatgcgcgccttgagcctggcgaacagttcggctggcgcgagcccctgatgctcttcgtccagatcatcctgatcgacaagaccggcttccatccgagtacgtgctcgctcgatgcgatgtttcgcttggtggtcgaatgggcaggtagccggatcaagcgtatgcagccgccgcattgcatcagccatgatggatactttctcggcaggagcaaggtgagatgacaggagatcctgccccggcacttcgcccaatagcagccagtcccttcccgcttcagtgacaacgtcgagcacagctgcgcaaggaacgcccgtcgtggccagccacgatagccgcgctgcctcgtcctgcagttcattcagggcaccggacaggtcggtcttgacaaaaagaaccgggcgcccctgcgctgacagccggaacacggcggcatcagagcagccgattgtctgttgtgcccagtcatagccgaatagcctctccacccaagcggccggagaacctgcgtgcaatccatcttgttcaatcatgcgaaacgatcctcatcctgtctcttgatcagatcttgatcccctgcgccatcagatccttggcggcaagaaagccatccagtttactttgcagggcttcccaaccttaccagagggcgccccagctggcaattccggttcgcttgctgtccataaaaccgcccagtctagctatcgccatgtaagcccactgcaagctacctgctttctctttgcgcttgcgttttcccttgtccagatagcccagtagctgacattcatccggggtcagcaccgtttctgcggactggctttctacgtgttccgcttcctttagcagcccttgcgccctgagtgcttgcggcagcgtgaagctaattcccatgtcagccgttaagtgttcctgtgtcactcaaaattgctttgagaggctctaagggcttctcagtgcgttacatccctggcttgttgtccacaaccgttaaaccttaaaagctttaaaagccttatatattcttttttttcttataaaacttaaaaccttagaggctatttaagttgctgatttatattaattttattgttcaaacatgagagcttagtacgtgaaacatgagagcttagtacgttagccatgagagcttagtacgttagccatgagggtttagttcgttaaacatgagagcttagtacgttaaacatgagagcttagtacgtgaaacatgagagcttagtacgtactatcaacaggttgaactgctgatcttcagatcctctacgccggacgcatcgtggccgttttccgctgcataaccctgcttcggggtcattatagcgattttttcggtatatccatcctttttcgcacgatatacaggattttgccaaagggttcgtgtagactttccttggtgtatccaacggcgtcagccgggcaggataggtgaagtaggcccacccgcgagcgggtgttccttcttcactgtcccttattcgcacctggcggtgctcaacgggaatcctgctctgcgaggctggccggctaccgccggcgtaacagatgagggcaagcggatggctgatgaaaccaagccaaccaggaagggcagcccacctatcaaggtgtactgccttccagacgaacgaagagcgattgaggaaaaggcggcggcggccggcatgagcctgtcggcctacctgctggccgtcggccagggctacaaaatcacgggcgtcgtggactatgagcacgtccgcgagctggcccgcatcaatggcgacctgggccgcctgggcggcctgctgaaactctggctcaccgacgacccgcgcacggcgcggttcggtgatgccacgatcctcgccctgctggcgaagatcgaagagaagcaggacgagcttggcaaggtcatgatgggcgtggtccgcccgagggcagagccatgacttttttagccgctaaaacggccggggggtgcgcgtgattgccaagcacgtccccatgcgctccatcaagaagagcgacttcgcggagctggtgaagtacatcaccgacgagcaaggcaagaccgaccaaagcggccatcgtgcctccccactcctgcagttcgggggcatggatgcgcggatagccgctgctggtttcctggatgccgacggatttgcactgccggtagaactccgcgaggtcgtccagcctcaggcagcagctgaaccaactcgcgaggggatcgagccccattcgccattcaggctgcgcaactgttgggaagggcgatcggtgcgggcctcttcgctattacgccagctggcgaaagggggatgtgctgcaaggcgattaagttgggtaacgccagggttttcccagtcacgacgttgtaaaacgacggccagtatagggataacagggtaatctgaattcgagctcggtaccctgaacgcttcgccagccaactgggccagactgagcgggctgcccgccagggggtggcccttgggcagcacggccaccagcgggtcctcgcacagcacctgctggtgaatcaccgggtcgtcgatgcgaatgcgcccgaagccaatgtcgatacgcccgcttttcagcgcctccacctgttgcaaggtggtcatttcgttcaggcccagttccagctcgctgtcctggcgcagctcgcggatcagctccggcagcacggtgtacagggtagagggcgcaaagccgatgcccagccactggcgctggccctggccgatgcggcgggtgttgtcgctgatgttctgcaactgctgcagcacggtgcaggtctgttcgtagaagaagcggccggcctcggtcagccgcagcggacgttcgcgcaccaccagcagggtcccgagctggtcctccagctggctgatctgccggctcaggggtggctgggcgatgtgcagcagctcggcggcgcgggtgaagttcagggtctcggccaagactttgaagtaacgcaggtggcgcagctccatcagacctccagggtatggtgggagattcatttgatattggacggtcgtcagggtctcgcgcaatccttcagcaatcaagtaaacgcatcactcgggcctgcaactgaaagcccgacctgacgggacctggcaacacatatgcagctcaaggccgacgaanaggaactggcccagcgcctgcagcgcgaaggcatctggcgtcacctgtggcgcattgccgggcattacgccaactacagcgtgttcgatgtgcccagcgtcgaggcattgcatgacacgctgatgcagctgccgctgttcccgtacatggatatcgaggtcgacggcctgtgtcggcatccctcgtctattcacagcgacgatcgctgattcgcacctgtatgcctgacaagaacaatacgaggtaagcacgatgaccgtgaaaatttcccacactgccgacattcaagccttcttcaaccgggtagctggcctggaccatgccgaaggaaacccgcgcttcaagcagatcattctgcgcgtgctgcaagacaccgcccgcctgatcgaagacctggagattaccgaggacgagttctggcacgccgtcgactacctcaaccgcctgggcggccgtaacgaggcaggcctgctggctgctggcctgggtatcgagcggggatcctctagagtcgacctgcaggcatgcaagcttctagggataacagggtaatccggcgtaatcatggtcatagctgtttcctgtgtgaaattgttatccgctcacaattccacacaacatacgagccggaagcataaagtgtaaagcctggggtgcctaatgagtgagctaactcacattaattgcgttgcgctcactgcccgctttccagtcgggaaacctgtcgtgccagctgcattaatgaatcggccaacgcgcggggagaggcggtttgcgtattggggggtgggcgaagaactccagcatgagatccccgcgctggaggatcatcca

SEQ ID NO: 54 - DNA, 4168 bp, artificial
  pEMG-deltapcaB
acaccgcgggcatgaccgccaagaacgccagctacgtgatgaccggggcgttgttcctgttcatggtggtgcagccgttcttcggcatgctgtccgaccgtatcggccggcgcaattcgatgctgctgttcggcggcctcggtaccctgtgcaccgtgccgctgctgatggcgctgaaaaccgtgaccagcccgatcatggccttcgtgctgatcagcctggccctgtgtatcgtgagtttctacacctcgatcagcggtctggtgaaggccgagatgttcccgccgcaggtgcgtgcactgggtgttggcctggcctacgcggtggccaacgcagcattcggcggttcggccgagtatgtggccctgggcctgaaaaccctggggatggaaaacactttctattggtacgtgacggcgatgatggcgattgccttcctgttcagcctgcgcctgccgaagcaggcggcgtacctgcaccatgatgattaaggacgctgcaggagaccgctgtggcgcacttgcaactggccgatggcgttttgaattaccagatcgatggcccggatgacgccccggtgctggtcctgtccaactcgctgggtaccgacctgggcatgtgggacacccagattccgctctggagtcagcacttccgggtgctgcgctatgacacccgtggtcacggcgcatcgctggtcactgaaggcccttacagcatcgaacagctgggccgcgacgtgctggccctgctcgatggcctggacattcaaaaggctcacttcgtcggcctgtcgatgggcggcctgatcggccagtggctgggtatccatgcaggtgagcgcctgcacagcctgaccctgtgcaacacggccgccaagatcgccaatgacgaggtgtggaacacccgtatcgacacggtactcaaaggcggccagcaggccatggtcgacctgcgcgatgcctccatcgcccgctggttcaccccgggctttgcccagggggatcctctagagtcgacctgcaggcatgcaagcttctagggataacagggtaatccggcgtaatcatggtcatagctgtttcctgtgtgaaattgttatccgctcacaattccacacaacatacgagccggaagcataaagtgtaaagcctggggtgcctaatgagtgagctaactcacattaattgcgttgcgctcactgcccgctttccagtcgggaaacctgtcgtgccagctgcattaatgaatcggccaacgcgcggggagaggcggtttgcgtattggggggtgggcgaagaactccagcatgagatccccgcgctggaggatcatccagccggcgtcccggaaaacgattccgaagcccaacctttcatagaaggcggcggtggaatcgaaatctcgtgatggcaggttgggcgtcgcttggtcggtcatttcgaaccccagagtcccgctcagaagaactcgtcaagaaggcgatagaaggcgatgcgctgcgaatcgggagcggcgataccgtaaagcacgaggaagcggtcagcccattcgccgccaagctcttcagcaatatcacgggtagccaacgctatgtcctgatagcggtccgccacacccagccggccacagtcgatgaatccagaaaagcggccattttccaccatgatattcggcaagcaggcatcgccatgggtcacgacgagatcctcgccgtcgggcatgcgcgccttgagcctggcgaacagttcggctggcgcgagcccctgatgctcttcgtccagatcatcctgatcgacaagaccggcttccatccgagtacgtgctcgctcgatgcgatgtttcgcttggtggtcgaatgggcaggtagccggatcaagcgtatgcagccgccgcattgcatcagccatgatggatactttctcggcaggagcaaggtgagatgacaggagatcctgccccggcacttcgcccaatagcagccagtcccttcccgcttcagtgacaacgtcgagcacagctgcgcaaggaacgcccgtcgtggccagccacgatagccgcgctgcctcgtcctgcagttcattcagggcaccggacaggtcggtcttgacaaaaagaaccgggcgcccctgcgctgacagccggaacacggcggcatcagagcagccgattgtctgttgtgcccagtcatagccgaatagcctctccacccaagcggccggagaacctgcgtgcaatccatcttgttcaatcatgcgaaacgatcctcatcctgtctcttgatcagatcttgatcccctgcgccatcagatccttggcggcaagaaagccatccagtttactttgcagggcttcccaaccttaccagagggcgccccagctggcaattccggttcgcttgctgtccataaaaccgcccagtctagctatcgccatgtaagcccactgcaagctacctgctttctctttgcgcttgcgttttcccttgtccagatagcccagtagctgacattcatccggggtcagcaccgtttctgcggactggctttctacgtgttccgcttcctttagcagcccttgcgccctgagtgcttgcggcagcgtgaagctaattcccatgtcagccgttaagtgttcctgtgtcactcaaaattgctttgagaggctctaagggcttctcagtgcgttacatccctggcttgttgtccacaaccgttaaaccttaaaagctttaaaagccttatatattcttttttttcttataaaacttaaaaccttagaggctatttaagttgctgatttatattaattttattgttcaaacatgagagcttagtacgtgaaacatgagagcttagtacgttagccatgagagcttagtacgttagccatgagggtttagttcgttaaacatgagagcttagtacgttaaacatgagagcttagtacgtgaaacatgagagcttagtacgtactatcaacaggttgaactgctgatcttcagatcctctacgccggacgcatcgtggccgttttccgctgcataaccctgcttcggggtcattatagcgattttttcggtatatccatcctttttcgcacgatatacaggattttgccaaagggttcgtgtagactttccttggtgtatccaacggcgtcagccgggcaggataggtgaagtaggcccacccgcgagcgggtgttccttcttcactgtcccttattcgcacctggcggtgctcaacgggaatcctgctctgcgaggctggccggctaccgccggcgtaacagatgagggcaagcggatggctgatgaaaccaagccaaccaggaagggcagcccacctatcaaggtgtactgccttccagacgaacgaagagcgattgaggaaaaggcggcggcggccggcatgagcctgtcggcctacctgctggccgtcggccagggctacaaaatcacgggcgtcgtggactatgagcacgtccgcgagctggcccgcatcaatggcgacctgggccgcctgggcggcctgctgaaactctggctcaccgacgacccgcgcacggcgcggttcggtgatgccacgatcctcgccctgctggcgaagatcgaagagaagcaggacgagcttggcaaggtcatgatgggcgtggtccgcccgagggcagagccatgacttttttagccgctaaaacggccggggggtgcgcgtgattgccaagcacgtccccatgcgctccatcaagaagagcgacttcgcggagctggtgaagtacatcaccgacgagcaaggcaagaccgaccaaagcggccatcgtgcctccccactcctgcagttcgggggcatggatgcgcggatagccgctgctggtttcctggatgccgacggatttgcactgccggtagaactccgcgaggtcgtccagcctcaggcagcagctgaaccaactcgcgaggggatcgagccccattcgccattcaggctgcgcaactgttgggaagggcgatcggtgcgggcctcttcgctattacgccagctggcgaaagggggatgtgctgcaaggcgattaagttgggtaacgccagggttttcccagtcacgacgttgtaaaacgacggccagtatagggataacagggtaatctgaattcgagctcggtaccc

SEQ ID NO: 55 - DNA, 4254 bp, artificial
  pEMG-pEM7
gccggcgtcccggaaaacgattccgaagcccaacctttcatagaaggcggcggtggaatcgaaatctcgtgatggcaggttgggcgtcgcttggtcggtcatttcgaaccccagagtcccgctcagaagaactcgtcaagaaggcgatagaaggcgatgcgctgcgaatcgggagcggcgataccgtaaagcacgaggaagcggtcagcccattcgccgccaagctcttcagcaatatcacgggtagccaacgctatgtcctgatagcggtccgccacacccagccggccacagtcgatgaatccagaaaagcggccattttccaccatgatattcggcaagcaggcatcgccatgggtcacgacgagatcctcgccgtcgggcatgcgcgccttgagcctggcgaacagttcggctggcgcgagcccctgatgctcttcgtccagatcatcctgatcgacaagaccggcttccatccgagtacgtgctcgctcgatgcgatgtttcgcttggtggtcgaatgggcaggtagccggatcaagcgtatgcagccgccgcattgcatcagccatgatggatactttctcggcaggagcaaggtgagatgacaggagatcctgccccggcacttcgcccaatagcagccagtcccttcccgcttcagtgacaacgtcgagcacagctgcgcaaggaacgcccgtcgtggccagccacgatagccgcgctgcctcgtcctgcagttcattcagggcaccggacaggtcggtcttgacaaaaagaaccgggcgcccctgcgctgacagccggaacacggcggcatcagagcagccgattgtctgttgtgcccagtcatagccgaatagcctctccacccaagcggccggagaacctgcgtgcaatccatcttgttcaatcatgcgaaacgatcctcatcctgtctcttgatcagatcttgatcccctgcgccatcagatccttggcggcaagaaagccatccagtttactttgcagggcttcccaaccttaccagagggcgccccagctggcaattccggttcgcttgctgtccataaaaccgcccagtctagctatcgccatgtaagcccactgcaagctacctgctttctctttgcgcttgcgttttcccttgtccagatagcccagtagctgacattcatccggggtcagcaccgtttctgcggactggctttctacgtgttccgcttcctttagcagcccttgcgccctgagtgcttgcggcagcgtgaagctaattcccatgtcagccgttaagtgttcctgtgtcactcaaaattgctttgagaggctctaagggcttctcagtgcgttacatccctggcttgttgtccacaaccgttaaaccttaaaagctttaaaagccttatatattcttttttttcttataaaacttaaaaccttagaggctatttaagttgctgatttatattaattttattgttcaaacatgagagcttagtacgtgaaacatgagagcttagtacgttagccatgagagcttagtacgttagccatgagggtttagttcgttaaacatgagagcttagtacgttaaacatgagagcttagtacgtgaaacatgagagcttagtacgtactatcaacaggttgaactgctgatcttcagatcctctacgccggacgcatcgtggccgttttccgctgcataaccctgcttcggggtcattatagcgattttttcggtatatccatcctttttcgcacgatatacaggattttgccaaagggttcgtgtagactttccttggtgtatccaacggcgtcagccgggcaggataggtgaagtaggcccacccgcgagcgggtgttccttcttcactgtcccttattcgcacctggcggtgctcaacgggaatcctgctctgcgaggctggccggctaccgccggcgtaacagatgagggcaagcggatggctgatgaaaccaagccaaccaggaagggcagcccacctatcaaggtgtactgccttccagacgaacgaagagcgattgaggaaaaggcggcggcggccggcatgagcctgtcggcctacctgctggccgtcggccagggctacaaaatcacgggcgtcgtggactatgagcacgtccgcgagctggcccgcatcaatggcgacctgggccgcctgggcggcctgctgaaactctggctcaccgacgacccgcgcacggcgcggttcggtgatgccacgatcctcgccctgctggcgaagatcgaagagaagcaggacgagcttggcaaggtcatgatgggcgtggtccgcccgagggcagagccatgacttttttagccgctaaaacggccggggggtgcgcgtgattgccaagcacgtccccatgcgctccatcaagaagagcgacttcgcggagctggtgaagtacatcaccgacgagcaaggcaagaccgaccaaagcggccatcgtgcctccccactcctgcagttcgggggcatggatgcgcggatagccgctgctggtttcctggatgccgacggatttgcactgccggtagaactccgcgaggtcgtccagcctcaggcagcagctgaaccaactcgcgaggggatcgagccccattcgccattcaggctgcgcaactgttgggaagggcgatcggtgcgggcctcttcgctattacgccagctggcgaaagggggatgtgctgcaaggcgattaagttgggtaacgccagggttttcccagtcacgacgttgtaaaacgacggccagtatagggataacagggtaatctgaattcgagctcggtaccctgggcgatgtgcagcagctcggcggcgcgggtgaagttcagggtctcggccaagactttgaagtaacgcaggtggcgcagctccatcagacctccagggtatggtgggagattcatttgatattggacggtcgtcagggtctcgcgcaatccttcagcaatcaagtaaacgcatcactcgggcctgcaactgaaagcccgacctgacgggacctggcaacacagctcaaggccgacgaaaaggaactggcccagcgcctgcagcgcgaaggcatctggcgtcacctgtggcgcattgccgggcattacgccaactacagcgtgttcgatgtgcccagcgtcgaggcattgcatgacacgctgatgcagctgccgctgttcccgtacatggatatcgaggtcgacggcctgtgtcggcatccctcgtctattcacagcgacgatcgctgattcgcacctgtatgcctgacaagaacaatacgaggtaagcacgttgttgacaattaatcatcggcatagtatatcggcatagtataatacgacaaggtgaggaactaaacccctaggttaaagaggagaaattaagcatgaccgtgaaaatttcccacactgccgacattcaagccttcttcaaccgggtagctggcctggaccatgccgaaggaaacccgcgcttcaagcagatcattctgcgcgtgctgcaagacaccgcccgcctgatcgaagacctggagattaccgaggacgagttctggcacgccgtcgactacctcaaccgcctgggcggccgtaacgaggcaggcctgctggctgctggcctgggtatcgagcacttcctcgacctgctgcaggatgccaaggatgccgaagccggccttggcggcggcaccccgcgcaccatcgaaggcccgttgtacgttgccggggcgccgctggcccagggcgaagcgcgcatggacgacggcactgacccaggcgtggtgatgttccttcagggccaggtgttcgatgccgacggcaagccgttggccggtgccaccgtcgacctgtggcacgccaatacccagggcacctattcgtacttcgaggggatcctctagagtcgacctgcaggcatgcaagcttctagggataacagggtaatccggcgtaatcatggtcatagctgtttcctgtgtgaaattgttatccgctcacaattccacacaacatacgagccggaagcataaagtgtaaagcctggggtgcctaatgagtgagctaactcacattaattgcgttgcgctcactgcccgctttccagtcgggaaacctgtcgtgccagctgcattaatgaatcggccaacgcgcggggagaggcggtttgcgtattggggggtgggcgaagaactccagcatgagatccccgcgctggaggatcatcca

SEQ ID NO: 56 - DNA, 40 bp, Artificial Sequence
  Primer sequence
caagcttaggaggaaaaacaaactggaagcggtgtcaaag

SEQ ID NO: 57 - DNA, 59 bp, Artificial Sequence
  Primer sequence
tcctcgcccttgctcaccatgcttaatttctcctctttgtggccggcattctatttgtc

SEQ ID NO: 58 - DNA, 21 bp, Artificial Sequence
  Primer sequence
aactggaagcggtgtcaaagc

SEQ ID NO: 59 - DNA, 19 bp, Artificial Sequence
  Primer sequence
gtggccggcattctatttg

SEQ ID NO: 60 - DNA, 40 bp, Artificial Sequence
  Primer sequence
caagcttaggaggaaaaacaccgcttcacagggaacacca

SEQ ID NO: 61 - DNA, 40 bp, Artificial Sequence
  Primer sequence
cctcgcccttgctcaccatcgatacaatcctccgcagaag

SEQ ID NO: 62 - DNA, 18 bp, Artificial Sequence
  Primer sequence
ccgcttcacagggaacac

SEQ ID NO: 63 - DNA, 21 bp, Artificial Sequence
  Primer sequence
cgatacaatcctccgcagaag

SEQ ID NO: 64 - DNA, 40 bp, Artificial Sequence
  Primer sequence
caagcttaggaggaaaaacagaaggaccggggccgcgcaa

SEQ ID NO: 65 - DNA, 40 bp, Artificial Sequence
  Primer sequence
tcctcgcccttgctcaccattgtcgatctctcccaaattg

SEQ ID NO: 66 - DNA, 40 bp, Artificial Sequence
  Primer sequence
tgaattcgagctcggtacccacaccgcgggcatgaccgcc

SEQ ID NO: 67 - DNA, 40 bp, Artificial Sequence
  Primer sequence
gtgcgccacagcggtctcctgcagcgtccttaatcatcat

SEQ ID NO: 68 - DNA, 40 bp, Artificial Sequence
  Primer sequence
atgatgattaaggacgctgcaggagaccgctgtggcgcac

SEQ ID NO: 69 - DNA, 40 bp, Artificial Sequence
  Primer sequence
gtcgactctagaggatccccctgggcaaagcccggggtga

SEQ ID NO: 70 - DNA, 45 bp, Artificial Sequence
  Primer sequence
taatctgaattcgagctcggtaccccgttggccggtgccaccgtc

SEQ ID NO: 71 - DNA, 50 bp, Artificial Sequence
  Primer sequence
gttcacggtcatgcttaatttctcctcttttcagccctcctgcaacgccc

SEQ ID NO: 72 - DNA, 20 bp, Artificial Sequence
  Primer sequence
gttcgaggttatgtcactgt

SEQ ID NO: 73 - DNA, 47 bp, Artificial Sequence
  Primer sequence
tgcaggtcgactctagaggatccccggcgggcagatcctgtgcgtag

SEQ ID NO: 74 - DNA, 45 bp, Artificial Sequence
  Primer sequence
gggctgaaaagaggagaaattaagcatgaccgtgaacatttccca

SEQ ID NO: 75 - DNA, 45 bp, Artificial Sequence
  Primer sequence
aaatcacagtgacataacctcgaactcaggcctcctgcaaagctc

SEQ ID NO: 76 - DNA, 45 bp, Artificial Sequence
  Primer sequence
taatctgaattcgagctcggtaccccgcgcctgaacgccgggcag

SEQ ID NO: 77 - DNA, 45 bp, Artificial Sequence
  Primer sequence
tctcccaccataccctggaggtctgacacaccatgcccacagggg

SEQ ID NO: 78 - DNA, 45 bp, Artificial Sequence
  Primer sequence
gccgcgagctttgcaggaggcctgatcatatggcctgttgctcga

SEQ ID NO: 79 - DNA, 45 bp, Artificial Sequence
  Primer sequence
tgcaggtcgactctagaggatcccctgaccaccttgcaacaggtg

SEQ ID NO: 80 - DNA, 20 bp, Artificial Sequence
  Primer sequence
cagacctccagggtatggtg

SEQ ID NO: 81 - DNA, 20 bp, Artificial Sequence
  Primer sequence
tcaggcctcctgcaaagctc

SEQ ID NO: 82 - DNA, 40 bp, Artificial Sequence
  Primer sequence
gtcgactctagaggatcccctcagccctcctgcaacgccc

SEQ ID NO: 83 - DNA, 20 bp, Artificial Sequence
  Primer sequence
atgaccgtgaaaatttccca

SEQ ID NO: 84 - DNA, 40 bp, Artificial Sequence
  Primer sequence
atatgtcgagctcggtacccgaaggaccggggccgcgcaa

SEQ ID NO: 85 - DNA, 40 bp, Artificial Sequence
  Primer sequence
tgggaaattttcacggtcattgtcgatctctcccaaattg

SEQ ID NO: 86 - DNA, 20 bp, Artificial Sequence
  Primer sequence
cgcgaattgcaagctgatcc

SEQ ID NO: 87 - DNA, 20 bp, Artificial Sequence
  Primer sequence
ctctcatccgccaaaacagc

SEQ ID NO: 88 - DNA, 501 bp, Artificial Sequence
  Promoter sequence
ccgcttcacagggaacaccactcaggcggtagggctgggagcggtaccaaagcagccaggtttcaggtttgattgaggaaacttgagaaaacgcttggcactaggacggcaggcaggtagaatgccggccacgcttggaggggtccccgagcggccaaaggggacgggctgtaaatccgttgcgagagcctcgaaggttcgagtcctcctccccccaccagttttagcgagggccgcaagccccgcgggtatagtttagtggtaaagcctcagccttccaagctgataatgcgggctcggttcccactacccgctccaagcttaccggatcttgcacagggtgtttcgctcttgtagcccagtcggtagaacacacccctggtaagggtgaggtcagcggctcaagtccgcttaaggactccgtatggacagggcgggtatgaaagtatctgcctctgttctgtcagtgcaagactaccccttctgcggaggattgtatcg

SEQ ID NO: 89 - DNA, 118 bp, Artificial Sequence
  Promoter sequence
aactggaagcggtgtcaaagcagctaagtttcagatttgattgaaaaaatttgaaaaaacgcttgacactaggacggcagacaaatagaatgccggccacaaagaggagaaattaagc

SEQ ID NO: 90 - DNA, 118 bp, Artificial Sequence
  Promoter sequence
aactggaagcggtgtcaaagcagctaggtttcggattcggttgacaaagtctggagggacgcttgacgttagggcggtagacaaatagaatgccggccacaaagaggagaaattaagc

SEQ ID NO: 91 - DNA, 116 bp, Artificial Sequence
  Promoter sequence
aactggaagcggtgtcaaagtagctgagttcggatctgattgaagaaatttgaaaaaacgcttggcactaggacggcagacaaatagaatgccggccacaaagaggagaaattaag

SEQ ID NO: 92 - DNA, 118 bp, Artificial Sequence
  Promoter sequence
aactggaagcggtgtcaaagtggctaggcttcagatttggttggaaaggtctgagaaaacgcttgacgctagagcggcagacaaatagaatgccggccacaaagaggagaaattaagc

SEQ ID NO: 93 - DNA, 119 bp, Artificial Sequence
  Promoter sequence
aactggaagcggtgtcaaagcagctgagcttcagatctgatcgagaagactcggggaaacgcttgacaccaggacagcagacaaatagaattgccggccacaaagaggagaaattaagc

SEQ ID NO: 94 - DNA, 118 bp, Artificial Sequence
  Promoter sequence
aactggaagcggtgtcaaagcagctgagtttcagacccgattggaaaggtttgaaggagcgcttgacactaggacggcagacaaatagaatgccggccacaaagaggagaaattaagc

SEQ ID NO: 95 - DNA, 118 bp, Artificial Sequence
  Promoter sequence
acctggaagcggtgtcaaagcagctgagtttcaggcctggttaagagagcttggaaaaacgtttgacactggggcggcagacaaatagaatgccggccacaaagaggagaaattaagc

SEQ ID NO: 96 - DNA, 118 bp, Artificial Sequence
  Promoter sequence
aactggaagcggtgtcaaagcagctaagtctcaggtttgattgggaaagtttggaaaagcgcttgacactaggacggcagacaaatagaatgccggccacaaagaggagaaattaagc

SEQ ID NO: 97 - DNA, 118 bp, Artificial Sequence
  Promoter sequence
aactggaagcggtgtcaaagcagctaaaccccaggtccggttgaagaagtttgaaaaaacgcttgacaccagggcggcagacaaatagaatgccggccacaaagaggagaaattaagc

SEQ ID NO: 98 - DNA, 118 bp, Artificial Sequence
  Promoter sequence
aactggaagcggtgtcaaagcagctaagtttcagacttgattgagaaaacttgaagaaacgcttgacaccaggatggcagacaaatagaatgccggccacaaagaggagaaattaagc

SEQ ID NO: 99 - DNA, 119 bp, Artificial Sequence
  Promoter sequence
aactggaagcggtgtcaaagcagctaagtttcagacttgattgaaagaatttggggaaacgcttgacactaggacggcagacaaatagaatgccggccacaaagaggagaaattaagct

SEQ ID NO: 100 - DNA, 118 bp, Artificial Sequence
  Promoter sequence
aactggaagcggtgtcaaagcagctaagtctcaggtttgatcgggaaagtctggaaaagcacttgacactagggcggcagacaaatagaatgccggccacaaagaggagaaattaagc

SEQ ID NO: 101 - DNA, 244 bp, Artificial Sequence
  Promoter sequence
gaaggaccggggccgcgcaagcggccccggtttttttttggcctgatgaaaaattttctatctcgagccttgtaatcggatgtggcggcctcatgtatgtggtcaccgcaaggtttctggtggcaacaccagacattacacaggtggttcgctcacagcgggccacccccggcaacgccggacagcatcaaaaccgccggtgtcgaaccggccgatgaaaaccacaatttgggagagatcgaca

SEQ ID NO: 102 - DNA, 244 bp, Artificial Sequence
  Promoter sequence
gaaggaccggggccgcgcaagcggccccggcttccctctggcctgatggagaatcctctaccccgagtcttgtggccgagtgcggcggcctcacgtatgtggtcaccgcagggcttctggtggtaacatcagatactgcacaggtggtccgctcacagcgggccacccccggcaacgccggacagcatcagaaccgccggtgccggaccggccgatgagagccacaatttgggagagatcgaca

SEQ ID NO: 103 - DNA, 244 bp, Artificial Sequence
  Promoter sequence
gaaggaccggggccgcgcaagtggctccggtttccctttggcccggtgaaaagtcttctaccttgagccctgtaatcggatgtggtagcctcatgtacgtggccaccgcgggatttctggtgacaacaccaggcatcacgcaggtggttcactcacagtgggccacccccggcaacgtcagacggcatcggaaccgccggtgtcgaaccggccgatgaaaaccacaatttgggagagatcgaca

SEQ ID NO: 104 - DNA, 244 bp, Artificial Sequence
  Promoter sequence
gaaggaccggggccgcgcaagtggctccggtttccctttggcccggtgaaaagtcttctaccttgagccctgtaatcggatgtggtagcctcatgtacgtggccaccgcgggatttctggtggcaacaccaggcatcacgcaggtggttcactcacagtgggccacccccggcaacgtcggacagcatcggaaccgccggtgtcgaaccggccgatgaaaaccgcaatttgggagagatcgaca

SEQ ID NO: 105 - DNA, 244 bp, Artificial Sequence
  Promoter sequence
gaaggaccggggccgcgcaagtggctccggtttccctttggcccggtgagaagtcttctaccttgagccctgtgatcggatgtggtagcctcatgtacgtggccaccgcgggatttctggtggcaacaccaggcatcacgcaggtggttcactcacagtgggccacccccggcaacgtcggacagcatcggaaccgccggtgtcgaaccggccgatgaaaaccacaatttgggagagatcgaca

SEQ ID NO: 106 - DNA, 4263 bp, Artificial Sequence
  Plasmid
ttaattaaagcggataacaatttcacacaggaggccgcctaggccgcggccgcgcgaattcgagctcggtacccggggatcctctagagtcgacctgcaggcatgcaagcttaggaggaaaaacatatggtgagcaagggcgaggaggataacatggccatcatcaaggagttcatgcgcttcaaggtgcacatggagggctccgtgaacggccacgagttcgagatcgagggcgagggcgagggccgcccctacgagggcacccagaccgccaagctgaaggtgaccaagggtggccccctgcccttcgcctgggacatcctgtcccctcagttcatgtacggctccaaggcctacgtgaagcaccccgccgacatccccgactacttgaagctgtccttccccgagggcttcaagtgggagcgcgtgatgaacttcgaggacggcggcgtggtgaccgtgacccaggactcctccctgcaagacggcgagttcatctacaaggtgaagctgcgcggcaccaacttcccctccgacggccccgtaatgcagaagaagaccatgggctgggaggcctcctccgagcggatgtaccccgaggacggcgccctgaagggcgagatcaagcagaggctgaagctgaaggacggcggccactacgacgctgaggtcaagaccacctacaaggccaagaagcccgtgcagctgcccggcgcctacaacgtcaacatcaagttggacatcacctcccacaacgaggactacaccatcgtggaacagtacgaacgcgccgagggccgccactccaccggcggcatggacgagctgtacaagtaaactagtcttggactcctgttgatagatccagtaatgacctcagaactccatctggatttgttcagaacgctcggttgccgccgggcgttttttattggtgagaatccaggggtccccaataattacgatttaaatttgtgtctcaaaatctctgatgttacattgcacaagataaaaatatatcatcatgaacaataaaactgtctgcttacataaacagtaatacaaggggtgttatgagccatattcagcgtgaaacgagctgtagccgtccgcgtctgaacagcaacatggatgcggatctgtatggctataaatgggcgcgtgataacgtgggtcagagcggcgcgaccatttatcgtctgtatggcaaaccggatgcgccggaactgtttctgaaacatggcaaaggcagcgtggcgaacgatgtgaccgatgaaatggtgcgtctgaactggctgaccgaatttatgccgctgccgaccattaaacattttattcgcaccccggatgatgcgtggctgctgaccaccgcgattccgggcaaaaccgcgtttcaggtgctggaagaatatccggatagcggcgaaaacattgtggatgcgctggccgtgtttctgcgtcgtctgcatagcattccggtgtgcaactgcccgtttaacagcgatcgtgtgtttcgtctggcccaggcgcagagccgtatgaacaacggcctggtggatgcgagcgattttgatgatgaacgtaacggctggccggtggaacaggtgtggaaagaaatgcataaactgctgccgtttagcccggatagcgtggtgacccacggcgattttagcctggataacctgattttcgatgaaggcaaactgattggctgcattgatgtgggccgtgtgggcattgcggatcgttatcaggatctggccattctgtggaactgcctgggcgaatttagcccgagcctgcaaaaacgtctgtttcagaaatatggcattgataatccggatatgaacaaactgcaatttcatctgatgctggatgaatttttctaataattaattggaccgcggtccgcgcgttgtccttttccgctgcataaccctgcttcggggtcattatagcgattttttcggtatatccatcctttttcgcacgatatacaggattttgccaaagggttcgtgtagactttccttggtgtatccaacggcgtcagccgggcaggataggtgaagtaggcccacccgcgagcgggtgttccttcttcactgtcccttattcgcacctggcggtgctcaacgggaatcctgctctgcgaggctggccgtaggccggccgataatctcatgaccaaaatcccttaacgtgagttttcgttccactgagcgtcagaccccgtagaaaagatcaaaggatcttcttgagatcctttttttctgcgcgtaatctgctgcttgcaaacaaaaaaaccaccgctaccagcggtggtttgtttgccggatcaagagctaccaactctttttccgaaggtaactggcttcagcagagcgcagataccaaatactgttcttctagtgtagccgtagttaggccaccacttcaagaactctgtagcaccgcctacatacctcgctctgctaatcctgttaccagtggctgctgccagtggcgataagtcgtgtcttaccgggttggactcaagacgatagttaccggataaggcgcagcggtcgggctgaacggggggttcgtgcacacagcccagcttggagcgaacgacctacaccgaactgagatacctacagcgtgagctatgagaaagcgccacgcttcccgaagggagaaaggcggacaggcatccggtaagcggcagggtcggaacaggagagcgcacgagggagcttccagggggaaacgcctggtatctttatagtcctgtcgggtttcgccacctctgacttgagcgtcgatttttgtgatgctcgtcaggggggcggagcctatggaaaaacgccagcaacgcggccgtgaaaggcaggccggtccgtggtggccacggcctctaggccagatccagcggcatctgggttagtcgagcgcgggccgcttcccatgtctcaccagggcgagcctgtttcgcgatctcagcatctgaaatcttcccggccttgcgcttcgctggggccttacccaccgccttggcgggcttcttcggtccaaaactgaacaacagatgtgtgaccttgcgcccggtctttcgctgcgcccactccacctgtagcgggctgtgctcgttgatctgcgtcacggctggatcaagcactcgcaacttgaagtccttgatcgagggataccggccttccagttgaaaccactttcgcagctggtcaatttctatttcgcgctggccgatgctgtcccattgcatgagcagctcgtaaagcctgatcgcgtgggtgctgtccatcttggccacgtcagccaaggcgtatttggtgaactgtttggtgagttccgtcaggtacggcagcatgtctttggtgaacctgagttctacacggccctcaccctcccggtagatgattgtttgcacccagccggtaatcatcacactcggtcttttccccttgccattgggctcttgggttaaccggacttcccgccgtttcaggcgcagggccgcttctttgagctggttgtaggaagattcgatagggacacccgccatcgtcgctatgtcctccgccgtcactgaatacatcacttcatcggtgacaggctcgctcctcttcacctggctaatacaggccagaacgatccgctgttcctgaacactgaggcgatacgcggcctcgaccagggcattgcttttgtaaaccattgggggtgaggccacgttcgacattccttgtgtataaggggacactgtatctgcgtcccacaatacaacaaatccgtccctttacaacaacaaatccgtcccttcttaacaacaaatccgtcccttaatggcaacaaatccgtccctttttaaactctacaggccacggattacgtggcctgtagacgtcctaaaaggtttaaaagggaaaaggaagaaaagggtggaaacgcaaaaaacgcaccactacgtggccccgttggggccgcatttgtgcccctgaaggggcgggggaggcgtctgggcaatccccgttttaccagtcccctatcgccgcctgagagggcgcaggaagcgagtaatcagggtatcgaggcggattcacccttggcgtccaaccagcggcaccagcggcgcctgagaggggcgcgcccagctgtctagggcggcggatttgtcctactcaggagagcgttcaccgacaaacaacagataaaacgaaaggcccagtctttcgactgagcctttcgttttatttgatgcct

SEQ ID NO: 107 - DNA, 5293 bp, Artificial Sequence
  Plasmid
tatgtcgagctcggtacccggggatcctctagagtcgacctgcaggcatgcaagcttggctgttttggcggatgagagaagattttcagcctgatacagattaaatcagaacgcagaagcggtctgataaaacagaatttgcctggcggcagtagcgcggtggtcccacctgaccccatgccgaactcagaagtgaaacgccgtagcgccgatggtagtgtggggtctccccatgcgagagtagggaactgccaggcatcaaataaaacgaaaggctcagtcgaaagactgggcctttcgttttatctgttgtttgtcggtgaacgctctcctgagtaggacaaatccgccgggagcggatttgaacgttgcgaagcaacggcccggagggtggcgggcaggacgcccgccataaactgccaggcatcaaattaagcagaaggccatcctgacggatggcctttttgcgtttctacaaactcttttgtttatttttctaaatacattcaaatatgtatccgctcatgagacaataaccctgataaatgcttcaataatattgaaaaaggaagagtatgagtattcaacatttccgtgtcgcccttattcccttttttgcggcattttgccttcctgtttttgctcacccagaaacgctggtgaaagtaaaagatgctgaagatcagttgggtgcacgagtgggttacatcgaactggatctcaacagcggtaagatccttgagagttttcgccccgaagaacgttttccaatgatgagcacttttaaagttctgctatgtggcgcggtattatcccgtgttgacgccgggcaagagcaactcggtcgccgcatacactattctcagaatgacttggttgagtactcaccagtcacagaaaagcatcttacggatggcatgacagtaagagaattatgcagtgctgccataaccatgagtgataacactgcggccaacttacttctgacaacgatcggaggaccgaaggagctaaccgcttttttgcacaacatgggggatcatgtaactcgccttgatcgttgggaaccggagctgaatgaagccataccaaacgacgagcgtgacaccacgatgcctgtagcaatggcaacaacgttgcgcaaactattaactggcgaactacttactctagcttcccggcaacaattaatagactggatggaggcggataaagttgcaggaccacttctgcgctcggcccttccggctggctggtttattgctgataaatctggagccggtgagcgtgggtctcgcggtatcattgcagcactggggccagatggtaagccctcccgtatcgtagttatctacacgacggggagtcaggcaactatggatgaacgaaatagacagatcgctgagataggtgcctcactgattaagcattggtaactgtcagaccaagtttactcatatatactttagattgatttaaaacttcatttttaatttaaaaggatctaggtgaagatcctttttgataatctcatgaccaaaatcccttaacgtgagttttcgttccactgagcgtcagaccccgtagaaaagatcaaaggatcttcttgagatcctttttttctgcgcgtaatctgctgcttgcaaacaaaaaaaccaccgctaccagcggtggtttgtttgccggatcaagagctaccaactctttttccgaaggtaactggcttcagcagagcgcagataccaaatactgtccttctagtgtagccgtagttaggccaccacttcaagaactctgtagcaccgcctacatacctcgctctgctaatcctgttaccagtggctgctgccagtggcgataagtcgtgtcttaccgggttggactcaagacgatagttaccggataaggcgcagcggtcgggctgaacggggggttcgtgcacacagcccagcttggagcgaacgacctacaccgaactgagatacctacagcgtgagctatgagaaagcgccacgcttcccgaagggagaaaggcggacaggtatccggtaagcggcagggtcggaacaggagagcgcacgagggagcttccagggggaaacgcctggtatctttatagtcctgtcgggtttcgccacctctgacttgagcgtcgatttttgtgatgctcgtcaggggggcggagcctatggaaaaacgccagcaacgcggcctttttacggttcctggccttttgctggccttttgctcacatgttctttcctgcgttatcccctgattctgtggataaccgtattaccgcctttgagtgagctgataccgctcgccgcagccgaacgaccgagcgcagcgagtcagtgagcgaggaagcggaagagcgcctgatgcggtattttctccttacgcatctgtgcggtatttcacaccgcatacggtgcactctcagtacaatctgctctgatgccgcatagttaagccagtatacactccgctatcgctacgtgactgggtcatggctgcgccccgacacccgccaacacccgctgacgcgccctgacgggcttgtctgctcccggcatccgcttacagacaagctgtgaccgtctccgggagctgcatgtgtcagaggttttcaccgtcatcaccgaaacgcgcgaggcagctgcggtaaagctcatcagcgtggtcgtgaagcgattcacagatgtctgcctgttcatccgcgtccagctcgttgagtttctccagaagcgttaatgtctggcttctgataaagcgggccatgttaagggcggttttttcctgtttggtcacttgatgcctccgtgtaagggggaatttctgttcatgggggtaatgataccgatgaaacgagagaggatgctcacgatacgggttactgatgatgaacatgcccggttactggaacgttgtgagggtaaacaactggcggtatggatgcggcgggaccagagaaaaatcactcagggtcaatgccagcgcttcgttaatacagatgtaggtgttccacagggtagccagcagcatcctgcgatgcagatccggaacataatggtgcagggcgctgacttccgcgtttccagactttacgaaacacggaaaccgaagaccattcatgttgttgctcaggtcgcagacgttttgcagcagcagtcgcttcacgttcgctcgcgtatcggtgattcattctgctaaccagtaaggcaaccccgccagcctagccgggtcctcaacgacaggagcacgatcatgcgcacccgtggccaggacccaacgctgcccgagatgcgccgcgtgcggctgctggagatggcggacgcgatggatatgttctgccaagggttggtttgcgcattcacagttctccgcaagaattgattggctccaattcttggagtggtgaatccgttagcgaggtgccgccggcttccattcaggtcgaggtggcccggctccatgcaccgcgacgcaacgcggggaggcagacaaggtatagggcggcgcctacaatccatgccaacccgttccatgtgctcgccgaggcggcataaatcgccgtgacgatcagcggtccagtgatcgaagttaggctggtaagagccgcgagcgatccttgaagctgtccctgatggtcgtcatctacctgcctggacagcatggcctgcaacgcgggcatcccgatgccgccggaagcgagaagaatcataatggggaaggccatccagcctcgcgtcgcgaacgccagcaagacgtagcccagcgcgtcggccagcttgcaattcgcgctaacttacattaattgcgttgcgctcactgcccgctttccagtcgggaaacctgtcgtgccagctgcattaatgaatcggccaacgcgcggggagaggcggtttgcgtattgggcgccagggtggtttttcttttcaccagtgagacgggcaacagctgattgcccttcaccgcctggccctgagagagttgcagcaagcggtccacgtggtttgccccagcaggcgaaaatcctgtttgatggtggttaacggcgggatataacatgagctgtcttcggtatcgtcgtatcccactaccgagatatccgcaccaacgcgcagcccggactcggtaatggcgcgcattgcgcccagcgccatctgatcgttggcaaccagcatcgcagtgggaacgatgccctcattcagcatttgcatggtttgttgaaaaccggacatggcactccagtcgccttcccgttccgctatcggctgaatttgattgcgagtgagatatttatgccagccagccagacgcagacgcgccgagacagaacttaatgggcccgctaacagcgcgatttgctggtgacccaatgcgaccagatgctccacgcccagtcgcgtaccgtcttcatgggagaaaataatactgttgatgggtgtctggtcagagacatcaagaaataacgccggaacattagtgcaggcagcttccacagcaatggcatcctggtcatccagcggatagttaatgatcagcccactgacgcgttgcgcgagaagattgtgcaccgccgctttacaggcttcgacgccgcttcgttctaccatcgacaccaccacgctggcacccagttgatcggcgcgagatttaatcgccgcgacaatttgcgacggcgcgtgcagggccagactggaggtggcaacgccaatcagcaacgactgtttgcccgccagttgttgtgccacgcggttgggaatgtaattcagctccgccatcgccgcttccactttttcccgcgttttcgcagaaacgtggctggcctggttcaccacgcgggaaacggtctgataagagacaccggcatactctgcgacatcgtataacgttactggtttcacattcaccaccctgaattgactctcttccgggcgctatcatgccataccgcgaaaggttttgcaccattcgatggtgtcaacgtaaatgccgcttcgccttcgcgcgcgaattgcaagctgatccgggcttatcgactgcacggtgcaccaatgcttctggcgtcaggcagccatcggaagctgtggtatggctgtgcaggtcgtaaatcactgcataattcgtgtcgctcaaggcgcactcccgttctggataatgttttttgcgccgacatcataacggttctggcaaatattctgaaatgagctgttgacaattaatcatcggctcgtataatgtgtggaattgtgagcggataacaatttcacacaggagatataca

SEQ ID NO: 108 - protein, 285 aa, Corynebacterium glutamicum
MTSAEQIVDPTAHDSGNKATDKFKANRVSSDTSKERANAIYVDLLAAIAQVAHKHEVTYEEYAVLKQWMIDVGEYGEWPLWLDVFVEHEIEEINYNRHDYTGTKGSIEGPYYVENSPKLPWDAEMPMRDKDRACTPLIFEGQVTDLDGNGLDGAEVELWHADEDGYYSQFAPGIPEWNLRGTIVTDEEGRYKIKTLQPAPYQIPHDGPTGWFIESYGGHPWRPAHLHLRVSHPGYRTITTQLYFEGGEWVENDVATAVKPELVLHPETGEDGNHVHYPFVLDKED

SEQ ID NO: 109 - protein, 373 aa, Corynebacterium glutamicum
MSDLTIQKVESRILDVPLIRPHGFATTTSTEQHILLVSVHLENGVIGYGEGVVPGGPWWGGESVETMKALVDGYLAPVLIGRAVSELAGIMADLERVVARARYAKAAVDVAMHDAWARSLNVPVRDLLGGTVRDKVDVTWALGVLPLDVAVAEIEERIEEFGNRSFKLKMGAGDPAEDTRRVAELAREVGDRVSLRIDINARWDRRTALHYLPILAEAGVELFEQPTPADDLETLREITRRTNVSVMADESVWTPAEALAVVKAQAADVIALKTTKHGGLLESKKIAAIAEAGGLACHGATSLEGPIGTAASLQFAASTKAISYGTELFGPQLLKDTYIVQEFEYKDGQVAIPQGPGLGVDVDMDKVNFYTRK

SEQ ID NO: 110 - DNA, 47 bp, artificial
  oligonucleotide primer
ttaacaattgggatcctctagacccactccagagcattggggtgttt

SEQ ID NO: 111 - DNA, 23 bp, artificial
  oligonucleotide primer
aggtccaatcggcaccgcagcat

SEQ ID NO: 112 - DNA, 48 bp, artificial
  oligonucleotide primer
ggatgctgcggtgccgattggaccctcaagcgccttcatggtctcaac

SEQ ID NO: 113 - DNA, 45 bp, artificial
  oligonucleotide primer
gcagcccgctagcgatttaaatccctgggcacccatggcgcccag

SEQ ID NO: 114 - DNA, 40 bp, artificial
  oligonucleotide primer
aattgggatcctctagacccacgattccctcttcagggcg

SEQ ID NO: 115 - DNA, 45 bp, artificial
  oligonucleotide primer
cattcgcagggtaacggccagtcatactcctagagactttggggg

SEQ ID NO: 116 - DNA, 40 bp, artificial
  oligonucleotide primer
aaagtctctaggagtatgactggccgttaccctgcgaatg

SEQ ID NO: 117 - DNA, 44 bp, artificial
  oligonucleotide primer
atctgttcagctgaagtcattgtatgtcctcctggacttcgtgg

SEQ ID NO: 118 - DNA, 42 bp, artificial
  oligonucleotide primer
gaagtccaggaggacatacaatgacttcagctgaacagatcg

SEQ ID NO: 119 - DNA, 41 bp, artificial
  oligonucleotide primer
ccgctagcgatttaaatccctagtatccgtcctcatctgcg

SEQ ID NO: 120 - DNA, 24 bp, artificial
  oligonucleotide primer
attgtctgttgtgcccagtcatag

SEQ ID NO: 121 - DNA, 20 bp, artificial
  oligonucleotide primer
aataatagtgaacggcaggt

SEQ ID NO: 122 - protein, 281 aa, Amycolatopsis sp.
MTATHHAPAAAESGASATARFKSDKFAAVADTPKERVSLLAREVLSAVHETIRKHKVTYDEYNALKAWLIQVGEDGEWPLFLDVWVEHVVEEVATSHRKGNKGTIEGPYYVPGAPEQGSRGSVPMREGEGGTPLVWTGRVTSVDGTPLKDAKVELWHADADGLYSQFAPGIPEWNLRGTFSVEEDGSFEIHTVRPAPYQIPTDGACGKLIAAAGWHAWRPAHLHVKVSAPGHELLTAQLYFPGDEHNDDDIASAVKPELVLDPKPSDGGETVTYDFVLDPA

SEQ ID NO: 123 - protein, 375 aa, Amycolatopsis sp.
MSATLDRVSRVRISSVTLPLATPISDAKVLTGRQKPMTEVAMLFAEITTENGLEGVGFSYSKRAGGPGQFAHAREIAPALLGEDPSDIAKIWDKLVWAGASVGRSGLSVQAIAAFDVALWDLKAKRAGLPLAKLLGAHRDSVRCYNTSGGFLHAPIEEVVERAAESVDRGIGGIKIKVGHPSHEVDLARVTAVREKIGDVPLMVDANQQWDRAAARRMCRALEPLDLVWIEEPLDAYDFEGHAQLSAAFDTPIATGEMLASAGEHAELIRARGADIVQPDAPRVGGITQFLKVMALADHAHLGLAPHFAMEVHIHLAAAYPREPWVEHFEWLDPLFDEHLEISGGRMHLSGRPGLGVTISEQARAWTVARDEVRV

SEQ ID NO: 124 - protein, 425 aa, Amycolatopsis sp.
MARIVALHTHDVRFPTSQTLDGSDAMNPDPDYSAAYLRLVTDAGDGLEGHGFVFTIGRGNDVQVAALRALEGHLLGRDVETTLADLGGLWRELVHDSQLRWLGPEKGIMHMAIGAAVNALWDLRAKREGKPLWQLLSSLTPEEIVDLVDFRYLTDALTRDEALEILRSAQPGRAEREARLLSEGYPAYTTTPGWLGYDDDKLARLCREAVDDGFRQIKLKVGADLDEDLRRLRIAREVCGPDVRIAVDANQRWDVGDAIAWIERLRPFDLAWIEEPTSPDDILGHAAIAEAVAPIPVATGEHGANRVLFKQLLQAKALSVLQLDATRVAGVNENIAILLLAAKFGVRVCPHAGGVGLCEAVQHLAMFDFVAVSSTTEDRMIEFVDHLHEHFVTPVDVHSGRYFAPKAPGAGTEMHAASLQEYAHG

SEQ ID NO: 125 - protein, 367 aa, Amycolatopsis sp.
MKITRVEAIPFAIPYRKPLKFASGEVHVAEHVLVRVHTDDGIVGVAEAPPRPFTYGETQAGIIAVIEKIFAPQVVGLTLLERETMASRLARTVGNPAAKAAIDMAVWDALGRTLDVQVTELLGGYTDRMRVSHMLGFDEPAAMVAEAQRMRDEHGITTFKVKVGRRPVALDTAVVRALREGMGDDVELYVDGNRGWTASESAMAMKEMTDLGLLFAEELCPADDVLGRRWLVSQLDVPFIADESAVTPADVTREILAGSATAISIKTARTGFTHSQRVHHLAEGLGLEVVMGNQIDGQIGSACTVAFGASYALTSRRAGELSNFLDMSDDLLTEPLEIHDGELHIRPGAGLGIEIDPAKLDRYRQDR

SEQ ID NO: 126 - DNA, 38 bp, artificial
  oligonucleotide primer
gatccgcggccgcgcgcgatcacgaaccggcggatcag

SEQ ID NO: 127 - DNA, 39 bp, artificial
  oligonucleotide primer
aagggagtgggtccgtgtgaggttccgggcccgttcgcg

SEQ ID NO: 128 - DNA, 38 bp, artificial
  oligonucleotide primer
cgaacgggcccggaacctcacacggacccactcccttg

SEQ ID NO: 129 - DNA, 40 bp, artificial
  oligonucleotide primer
gacatgattacgaattcgatcgaccacgctcagcgccttc

SEQ ID NO: 130 - DNA, 40 bp, artificial
  oligonucleotide primer
gatccgcggccgcgcgcgatcgcccttgttcgggtagtag

SEQ ID NO: 131 - DNA, 37 bp, artificial
  oligonucleotide primer
gacatgattacgaattcgatgacgctccactcgtttc

SEQ ID NO: 132 - DNA, 45 bp, artificial
  oligonucleotide primer
cttgatatccgggggagtttcacatcggctgacctcgtgtggttg

SEQ ID NO: 133 - DNA, 50 bp, artificial
  oligonucleotide primer
cccccaaccacacgaggtcagccgatgtgaaactcccccggatatcaagg